European Patent Specification EP 3 826 667 B1, published April 17, 2024. Title: CLAUDIN6 ANTIBODIES AND METHODS OF TREATING CANCER. Applicant: THE REGENTS OF THE UNIVERSITY OF CALIFORNIA. The sequence listing filed with the application follows.

SEQUENCE LISTING (489 sequences)

SEQ ID NO: 1 - protein, 220 aa, Homo sapiens
  ref <308>: NCBI / NP_067018.2
  ref <309>: 2017-06-04
  ref <313>: (1)..(220)
MASAGMQILGVVLTLLGWVNGLVSCALPMWKVTAFIGNSIVVAQVVWEGLWMSCVVQSTGQMQCKVYDSLLALPQDLQAARALCVIALLVALFGLLVYLAGAKCTTCVEEKDSKARLVLTSGIVFVISGVLTLIPVCWTAHAIIRDFYNPLVAEAQKRELGASLYLGWAASGLLLLGGGLLCCTCPSGGSQGPSHYMARYSTSAPAISRGPSEYPTKNYV

SEQ ID NO: 2 - protein, 23 aa, Homo sapiens
WTAHAIIRDFYNPLVAEAQKREL

SEQ ID NO: 3 - protein, 13 aa, Homo sapiens
TAHAIIRDFYNPL

SEQ ID NO: 4 - protein, 10 aa, Homo sapiens
LVAEAQKREL

SEQ ID NO: 5 - protein, 220 aa, Homo sapiens
  ref <308>: NCBI / NP_001297.1
  ref <309>: 2017-07-10
  ref <313>: (1)..(220)
MSMGLEITGTALAVLGWLGTIVCCALPMWRVSAFIGSNIITSQNIWEGLWMNCVVQSTGQMQCKVYDSLLALPQDLQAARALIVVAILLAAFGLLVALVGAQCTNCVQDDTAKAKITIVAGVLFLLAALLTLVPVSWSANTIIRDFYNPVVPEAQKREMGAGLYVGWAAAALQLLGGALLCCSCPPREKKYTATKVVYSAPRSTGPGASLGTGYDRKDYV

SEQ ID NO: 6 - protein, 209 aa, Homo sapiens
  ref <308>: NCBI / NP_001296.1
  ref <309>: 2017-07-10
  ref <313>: (1)..(209)
MASMGLQVMGIALAVLGWLAVMLCCALPMWRVTAFIGSNIVTSQTIWEGLWMNCVVQSTGQMQCKVYDSLLALPQDLQAARALVIISIIVAALGVLLSVVGGKCTNCLEDESAKAKTMIVAGVVFLLAGLMVIVPVSWTAHNIIQDFYNPLVASGQKREMGASLYVGWAASGLLLLGGGLLCCNCPPRTDKPYSAKYSAARSAAASNYV

SEQ ID NO: 7 - protein, 217 aa, Homo sapiens
  ref <308>: NCBI / NP_066192.1
  ref <309>: 2017-04-15
  ref <313>: (1)..(217)
MASTGLELLGMTLAVLGWLGTLVSCALPLWKVTAFIGNSIVVAQVVWEGLWMSCVVQSTGQMQCKVYDSLLALPQDLQAARALCVIALLLALLGLLVAITGAQCTTCVEDEGAKARIVLTAGVILLLAGILVLIPVCWTAHAIIQDFYNPLVAEALKRELGASLYLGWAAAALLMLGGGLLCCTCPPPQVERPRGPRLGYSIPSRSGASGLDKRDYV

SEQ ID NO: 8 - protein, 7 aa, Artificial Sequence
  Synthetic peptide
SSVSSTY

SEQ ID NO: 9 - protein, 3 aa, Artificial Sequence
  Synthetic peptide
STS

SEQ ID NO: 10 - protein, 9 aa, Artificial Sequence
  Synthetic peptide
HQYHRSPLT

SEQ ID NO: 11 - protein, 8 aa, Artificial Sequence
  Synthetic peptide
GYTFTTYT

SEQ ID NO: 12 - protein, 8 aa, Artificial Sequence
  Synthetic peptide
INPSSGYT

SEQ ID NO: 13 - protein, 9 aa, Artificial Sequence
  Synthetic peptide
ANGDYYVAY

SEQ ID NO: 14 - protein, 6 aa, Artificial Sequence
  Synthetic peptide
ENIYSY

SEQ ID NO: 15 - protein, 3 aa, Artificial Sequence
  Synthetic peptide
NAK

SEQ ID NO: 16 - protein, 9 aa, Artificial Sequence
  Synthetic peptide
QHHYTVPWT

SEQ ID NO: 17 - protein, 8 aa, Artificial Sequence
  Synthetic peptide
GFTFSDYW

SEQ ID NO: 18 - protein, 10 aa, Artificial Sequence
  Synthetic peptide
IRLKSDNYAT

SEQ ID NO: 19 - protein, 8 aa, Artificial Sequence
  Synthetic peptide
NDGPPSGC

SEQ ID NO: 20 - protein, 6 aa, Artificial Sequence
  Synthetic peptide
ENIYSY

SEQ ID NO: 21 - protein, 3 aa, Artificial Sequence
  Synthetic peptide
NAK

SEQ ID NO: 22 - protein, 9 aa, Artificial Sequence
  Synthetic peptide
QHHYTVPWT

SEQ ID NO: 23 - protein, 8 aa, Artificial Sequence
  Synthetic peptide
GFTFSNYW

SEQ ID NO: 24 - protein, 10 aa, Artificial Sequence
  Synthetic peptide
IRLKSDNYAT

SEQ ID NO: 25 - protein, 8 aa, Artificial Sequence
  Synthetic peptide
NDGPPSGC

SEQ ID NO: 26 - protein, 11 aa, Artificial Sequence
  Synthetic peptide
QSLVHSDGNTY

SEQ ID NO: 27 - protein, 3 aa, Artificial Sequence
  Synthetic peptide
KVS

SEQ ID NO: 28 - protein, 9 aa, Artificial Sequence
  Synthetic peptide
SQSTHVPYT

SEQ ID NO: 29 - protein, 8 aa, Artificial Sequence
  Synthetic peptide
GYTFTSYT

SEQ ID NO: 30 - protein, 8 aa, Artificial Sequence
  Synthetic peptide
INPSSTYT

SEQ ID NO: 31 - protein, 10 aa, Artificial Sequence
  Synthetic peptide
SRGELGGFAY

SEQ ID NO: 32 - protein, 11 aa, Artificial Sequence
  Synthetic peptide
QSIVHSNGNTY

SEQ ID NO: 33 - protein, 3 aa, Artificial Sequence
  Synthetic peptide
KVS

SEQ ID NO: 34 - protein, 9 aa, Artificial Sequence
  Synthetic peptide
FQGSHVPFT

SEQ ID NO: 35 - protein, 8 aa, Artificial Sequence
  Synthetic peptide
GYIFTHYI

SEQ ID NO: 36 - protein, 8 aa, Artificial Sequence
  Synthetic peptide
INPYNDGT

SEQ ID NO: 37 - protein, 13 aa, Artificial Sequence
  Synthetic peptide
ARYYGYPYYSMDY

SEQ ID NO: 38 - protein, 12 aa, Artificial Sequence
  Synthetic peptide
QSLLNSRTRKNY

SEQ ID NO: 39 - protein, 3 aa, Artificial Sequence
  Synthetic peptide
WAS

SEQ ID NO: 40 - protein, 8 aa, Artificial Sequence
  Synthetic peptide
KQSYYLYT

SEQ ID NO: 41 - protein, 9 aa, Artificial Sequence
  Synthetic peptide
GYSITSGYY

SEQ ID NO: 42 - protein, 7 aa, Artificial Sequence
  Synthetic peptide
ISYDGGI

SEQ ID NO: 43 - protein, 10 aa, Artificial Sequence
  Synthetic peptide
ARFGKGAMDY

SEQ ID NO: 44 - protein, 7 aa, Artificial Sequence
  Synthetic peptide
SSVSSSY

SEQ ID NO: 45 - protein, 3 aa, Artificial Sequence
  Synthetic peptide
STS

SEQ ID NO: 46 - protein, 9 aa, Artificial Sequence
  Synthetic peptide
HQYHRSPPT

SEQ ID NO: 47 - protein, 8 aa, Artificial Sequence
  Synthetic peptide
GYSFTGYT

SEQ ID NO: 48 - protein, 8 aa, Artificial Sequence
  Synthetic peptide
INPYNGGT

SEQ ID NO: 49 - protein, 12 aa, Artificial Sequence
  Synthetic peptide
ARGVYDYDGFTY

SEQ ID NO: 50 - protein, 11 aa, Artificial Sequence
  Synthetic peptide
QSLVHSDGNTY

SEQ ID NO: 51 - protein, 3 aa, Artificial Sequence
  Synthetic peptide
KVS

SEQ ID NO: 52 - protein, 9 aa, Artificial Sequence
  Synthetic peptide
SQSTHVPYT

SEQ ID NO: 53 - protein, 8 aa, Artificial Sequence
  Synthetic peptide
GYTFTTYT

SEQ ID NO: 54 - protein, 8 aa, Artificial Sequence
  Synthetic peptide
INPRSGYS

SEQ ID NO: 55 - protein, 10 aa, Artificial Sequence
  Synthetic peptide
SRGELGGFAY

SEQ ID NO: 56 - protein, 6 aa, Artificial Sequence
  Synthetic peptide
QTIGTW

SEQ ID NO: 57 - protein, 3 aa, Artificial Sequence
  Synthetic peptide
AAA

SEQ ID NO: 58 - protein, 9 aa, Artificial Sequence
  Synthetic peptide
QQLYSIPRT

SEQ ID NO: 59 - protein, 8 aa, Artificial Sequence
  Synthetic peptide
GYRFTDYN

SEQ ID NO: 60 - protein, 8 aa, Artificial Sequence
  Synthetic peptide
INPNNGGT

SEQ ID NO: 61 - protein, 10 aa, Artificial Sequence
  Synthetic peptide
ARDYLYFFDC

SEQ ID NO: 62 - protein, 11 aa, Artificial Sequence
  Synthetic peptide
QSLVHSNGNTY

SEQ ID NO: 63 - protein, 3 aa, Artificial Sequence
  Synthetic peptide
KVS

SEQ ID NO: 64 - protein, 9 aa, Artificial Sequence
  Synthetic peptide
SQITHVPYT

SEQ ID NO: 65 - protein, 8 aa, Artificial Sequence
  Synthetic peptide
GYTFTDYS

SEQ ID NO: 66 - protein, 8 aa, Artificial Sequence
  Synthetic peptide
ISTETGEP

SEQ ID NO: 67 - protein, 10 aa, Artificial Sequence
  Synthetic peptide
TRGLWSSFAY

SEQ ID NO: 68 - protein, 10 aa, Artificial Sequence
  Synthetic peptide
KSVSTSGYSY

SEQ ID NO: 69 - protein, 3 aa, Artificial Sequence
  Synthetic peptide
LAS

SEQ ID NO: 70 - protein, 9 aa, Artificial Sequence
  Synthetic peptide
QHSRELPLT

SEQ ID NO: 71 - protein, 8 aa, Artificial Sequence
  Synthetic peptide
GFTFSSFG

SEQ ID NO: 72 - protein, 8 aa, Artificial Sequence
  Synthetic peptide
ISSDSRTI

SEQ ID NO: 73 - protein, 11 aa, Artificial Sequence
  Synthetic peptide
ARDYGRTYEAY

SEQ ID NO: 74 - protein, 6 aa, Artificial Sequence
  Synthetic peptide
QDIGGN

SEQ ID NO: 75 - protein, 3 aa, Artificial Sequence
  Synthetic peptide
STS

SEQ ID NO: 76 - protein, 9 aa, Artificial Sequence
  Synthetic peptide
LQRNAYPLT

SEQ ID NO: 77 - protein, 8 aa, Artificial Sequence
  Synthetic peptide
GFTFSSYA

SEQ ID NO: 78 - protein, 7 aa, Artificial Sequence
  Synthetic peptide
IRSGGTT

SEQ ID NO: 79 - protein, 12 aa, Artificial Sequence
  Synthetic peptide
AKVGGNPYPMDY

SEQ ID NO: 80 - protein, 7 aa, Artificial Sequence
  Synthetic peptide
SSISSNY

SEQ ID NO: 81 - protein, 3 aa, Artificial Sequence
  Synthetic peptide
RTS

SEQ ID NO: 82 - protein, 9 aa, Artificial Sequence
  Synthetic peptide
QQGSSIPLT

SEQ ID NO: 83 - protein, 8 aa, Artificial Sequence
  Synthetic peptide
GYAFSNYL

SEQ ID NO: 84 - protein, 8 aa, Artificial Sequence
  Synthetic peptide
INPGSGGT

SEQ ID NO: 85 - protein, 15 aa, Artificial Sequence
  Synthetic peptide
ARSYFGRSYPYTMDY

SEQ ID NO: 86 - protein, 10 aa, Artificial Sequence
  Synthetic peptide
QSVDYDGDNY

SEQ ID NO: 87 - protein, 3 aa, Artificial Sequence
  Synthetic peptide
AAS

SEQ ID NO: 88 - protein, 9 aa, Artificial Sequence
  Synthetic peptide
QQSNEDPFT

SEQ ID NO: 89 - protein, 8 aa, Artificial Sequence
  Synthetic peptide
GYTFTDYA

SEQ ID NO: 90 - protein, 8 aa, Artificial Sequence
  Synthetic peptide
ISTYSGNT

SEQ ID NO: 91 - protein, 13 aa, Artificial Sequence
  Synthetic peptide
ARRGDYSLYAMDY

SEQ ID NO: 92 - protein, 12 aa, Artificial Sequence
  Synthetic peptide
QSVLFSSNQKNY

SEQ ID NO: 93 - protein, 3 aa, Artificial Sequence
  Synthetic peptide
WAS

SEQ ID NO: 94 - protein, 8 aa, Artificial Sequence
  Synthetic peptide
HQYLSSRT

SEQ ID NO: 95 - protein, 8 aa, Artificial Sequence
  Synthetic peptide
GFTFSSFG

SEQ ID NO: 96 - protein, 8 aa, Artificial Sequence
  Synthetic peptide
ISSDSRTI

SEQ ID NO: 97 - protein, 11 aa, Artificial Sequence
  Synthetic peptide
ARDYGRTYEAY

SEQ ID NO: 98 - protein, 10 aa, Artificial Sequence
  Synthetic peptide
ESVDNYGISF

SEQ ID NO: 99 - protein, 3 aa, Artificial Sequence
  Synthetic peptide
AAS

SEQ ID NO: 100 - protein, 9 aa, Artificial Sequence
  Synthetic peptide
QQSKEVPLT

SEQ ID NO: 101 - protein, 8 aa, Artificial Sequence
  Synthetic peptide
GFPFSSSA

SEQ ID NO: 102 - protein, 7 aa, Artificial Sequence
  Synthetic peptide
INSDGNT

SEQ ID NO: 103 - protein, 13 aa, Artificial Sequence
  Synthetic peptide
TRNGDYRYDEFAY

SEQ ID NO: 104 - protein, 7 aa, Artificial Sequence
  Synthetic peptide
SSVSSSY

SEQ ID NO: 105 - protein, 3 aa, Artificial Sequence
  Synthetic peptide
STS

SEQ ID NO: 106 - protein, 9 aa, Artificial Sequence
  Synthetic peptide
HQYHRSPPT

SEQ ID NO: 107 - protein, 8 aa, Artificial Sequence
  Synthetic peptide
GYTFTGYW

SEQ ID NO: 108 - protein, 8 aa, Artificial Sequence
  Synthetic peptide
INPSTGYT

SEQ ID NO: 109 - protein, 12 aa, Artificial Sequence
  Synthetic peptide
AREGITTVLVDY

SEQ ID NO: 110 - protein, 12 aa, Artificial Sequence
  Synthetic peptide
QSVLFSSNQKNY

SEQ ID NO: 111 - protein, 3 aa, Artificial Sequence
  Synthetic peptide
WAS

SEQ ID NO: 112 - protein, 8 aa, Artificial Sequence
  Synthetic peptide
HQYLSSRT

SEQ ID NO: 113 - protein, 8 aa, Artificial Sequence
  Synthetic peptide
GYSFTGYN

SEQ ID NO: 114 - protein, 8 aa, Artificial Sequence
  Synthetic peptide
IDPYYGGS

SEQ ID NO: 115 - protein, 14 aa, Artificial Sequence
  Synthetic peptide
ARERSGYVFSAMDY

SEQ ID NO: 116 - protein, 12 aa, Artificial Sequence
  Synthetic peptide
QSVLFSSNQKNY

SEQ ID NO: 117 - protein, 3 aa, Artificial Sequence
  Synthetic peptide
WAS

SEQ ID NO: 118 - protein, 8 aa, Artificial Sequence
  Synthetic peptide
HQYLSSRT

SEQ ID NO: 119 - protein, 8 aa, Artificial Sequence
  Synthetic peptide
GYSFTGYT

SEQ ID NO: 120 - protein, 8 aa, Artificial Sequence
  Synthetic peptide
INPYNGVT

SEQ ID NO: 121 - protein, 16 aa, Artificial Sequence
  Synthetic peptide
TRDPLYYGYRDSTMDY

SEQ ID NO: 122 - protein, 11 aa, Artificial Sequence
  Synthetic peptide
QSLVHSDGNTY

SEQ ID NO: 123 - protein, 3 aa, Artificial Sequence
  Synthetic peptide
KVS

SEQ ID NO: 124 - protein, 9 aa, Artificial Sequence
  Synthetic peptide
SQSTHVPYT

SEQ ID NO: 125 - protein, 8 aa, Artificial Sequence
  Synthetic peptide
GYTFTSYT

SEQ ID NO: 126 - protein, 8 aa, Artificial Sequence
  Synthetic peptide
INPSSTYT

SEQ ID NO: 127 - protein, 10 aa, Artificial Sequence
  Synthetic peptide
SRGELGGFAY

SEQ ID NO: 128 - protein, 6 aa, Artificial Sequence
  Synthetic peptide
QGIRGN

SEQ ID NO: 129 - protein, 3 aa, Artificial Sequence
  Synthetic peptide
STS

SEQ ID NO: 130 - protein, 9 aa, Artificial Sequence
  Synthetic peptide
LQRNAYPLT

SEQ ID NO: 131 - protein, 8 aa, Artificial Sequence
  Synthetic peptide
GFTFSSFA

SEQ ID NO: 132 - protein, 7 aa, Artificial Sequence
  Synthetic peptide
IRSGGIT

SEQ ID NO: 133 - protein, 13 aa, Artificial Sequence
  Synthetic peptide
ARVSTATYYGMDY

SEQ ID NO: 134 - protein, 108 aa, Artificial Sequence
  Synthetic peptide
QIVLTQSPAIMSASLGERVTMTCTASSSVSSTYFHWYQQKPGSSPKLWIYSTSNLASGVPRRFSGSASGTSYSLTISSMEAEDAATYYCHQYHRSPLTFGAGTKLELK

SEQ ID NO: 135 - protein, 116 aa, Artificial Sequence
  Synthetic peptide
QVQLQQSAAELARPGASVKMSCKASGYTFTTYTMHWVKQRPGQGLEWIGFINPSSGYTDYNQKFKDRTTLTADKSSSTVYMQLSSLTSEDSAVYYCANGDYYVAYWGQGTLVTVSA

SEQ ID NO: 136 - protein, 107 aa, Artificial Sequence
  Synthetic peptide
DIQMTQSPASLSASVGETVTITCRISENIYSYLAWYQQKQGKSPQLLVYNAKILVEGVPSRFSGSGSGTQFSLKINSLQPEDFGNYYCQHHYTVPWTFGGGTKLEIK

SEQ ID NO: 137 - protein, 117 aa, Artificial Sequence
  Synthetic peptide
EVKLEESGGGLVQPGGSMKLSCVASGFTFSDYWMNWVRQSPEKGLEWVAQIRLKSDNYATHYAESVKGRFTISRDDSKRSVYLQMNNLRAEDTGTYYCNDGPPSGCWGQGTTLIVSS

SEQ ID NO: 138 - protein, 107 aa, Artificial Sequence; identical to SEQ ID NO: 136
  Synthetic peptide

SEQ ID NO: 139 - protein, 117 aa, Artificial Sequence
  Synthetic peptide
EVKLEESGGGLVQPGGSMKLSCVASGFTFSNYWMNWVRQSPEKGLEWVAQIRLKSDNYATHYAESVKGRFTISRDDSKRSVYLQMNNLRAEDTGTYYCNDGPPSGCWGQGTTLIVSS

SEQ ID NO: 140 - protein, 112 aa, Artificial Sequence
  Synthetic peptide
DVVMTQTPLSLPVSLGDQASISCRSSQSLVHSDGNTYLNWYLQKPGQSPKLLIYKVSNRFSGVPDRFSGSGSGTDFTLKIRRVEAEDLGVYFCSQSTHVPYTFGGGTKLEIK

SEQ ID NO: 141 - protein, 117 aa, Artificial Sequence
  Synthetic peptide
QVQLQQSGAELARPGASVKMSCKASGYTFTSYTMHWIKQRPGQGQEWIGYINPSSTYTHYIKKFKDKATLTADKSSSTAYMQLRSLTSEDSAVYYCSRGELGGFAYWGQGTLVTVSA

SEQ ID NO: 142 - protein, 112 aa, Artificial Sequence
  Synthetic peptide
DVLMTQTPLSLPVSLGDQPSISCRSSQSIVHSNGNTYLDWYLQKPGQSPKLLIYKVSNRFSGVPDRFSGSGSGTDFTLKISRVEAEDLGVYYCFQGSHVPFTFGSGTRLEIK

SEQ ID NO: 143 - protein, 120 aa, Artificial Sequence
  Synthetic peptide
EVQLQQSGPELVKPGASVKMSCKASGYIFTHYIMHWVKQKPGQGLEWIGCINPYNDGTKYNEKFKGKATLTSDKSSSTAYMELSSLTSEDSAVYYCARYYGYPYYSMDYWGQGTSVTVSS

SEQ ID NO: 144 - protein, 112 aa, Artificial Sequence
  Synthetic peptide
AIVMFQSPSSLVVSAGEKVTMSCKSSQSLLNSRTRKNYLAWYQQKPGQSPKLLIYWASTRESGVPDRFTGSGSGTDFTLTISSVQAEDLAVYYCKQSYYLYTFGGGTKLEIK

SEQ ID NO: 145 - protein, 117 aa, Artificial Sequence
  Synthetic peptide
DVQLQESGPGLVKSSQSLSLTCSVTGYSITSGYYWKWIRQFPGNKLEWMGYISYDGGINYNPSLKNRISITRDTSKNQFFLKLNSVTTEDTAKYYCARFGKGAMDYWGQGTSVTVSS

SEQ ID NO: 146 - protein, 108 aa, Artificial Sequence
  Synthetic peptide
QIVLTQSPAIMSASLGDRVTMTCTASSSVSSSYLHWYQQKPGSSPKLWIYSTSNLASGVPARFSGSGSGTSYSLTISSMEAEDAATYYCHQYHRSPPTFGSGTKLEIK

SEQ ID NO: 147 - protein, 119 aa, Artificial Sequence
  Synthetic peptide
EVQLQQSGPELVKPGASMKISCKASGYSFTGYTMNWVKQSHGKNLEWIGLINPYNGGTNYNQKFKGKATLTVDKSSSTAYMELLSLTSEDSAVYYCARGVYDYDGFTYWGQGTLVTVSA

SEQ ID NO: 148 - protein, 112 aa, Artificial Sequence
  Synthetic peptide
DVVMTQTPLSLPVSLGDQASISCRSSQSLVHSDGNTYLYWYLQKPGQSPKLLIYKVSNRFSGVPDRFSGSGSGTDFTLKISRVEAEDLGVYFCSQSTHVPYTFGGGTKLEIK

SEQ ID NO: 149 - protein, 117 aa, Artificial Sequence
  Synthetic peptide
QVQLQQSGAELARPGASVKMSCKASGYTFTTYTMHWLKQRPGQGLEWIGYINPRSGYSNYNQKFKDKATLTADKSSNTAYMQLNTLTSEDSKVYYCSRGELGGFAYWGQGTLVTVSA

SEQ ID NO: 150 - protein, 107 aa, Artificial Sequence
  Synthetic peptide
DIQMTQSPASQSASLGESVTITCLASQTIGTWLAWYQQKPGKSPQLLIYAAASLADGVPSRFSGSGSGTRFSFKISSLQAEDFVSYYCQQLYSIPRTFGGGTKLEIK

SEQ ID NO: 151 - protein, 117 aa, Artificial Sequence
  Synthetic peptide
EVQLQQSGPELVKPGASVKMSCKASGYRFTDYNMHWVKQSHGKSLEWIGYINPNNGGTNYNQNFKGKATLTVNKSSSTAYMELRSLTSEDSAAYYCARDYLYFFDCWGQGTTLTVSS

SEQ ID NO: 152 - protein, 112 aa, Artificial Sequence
  Synthetic peptide
DVVMTQTPLSLPVSLGDQASISCRASQSLVHSNGNTYLHWFLQKPGQSPKLLIYKVSNRFSGVPDRFSGSGSRTDFTLKISRVEAEDLGVYFCSQITHVPYTFGGGTKLEIK

SEQ ID NO: 153 - protein, 117 aa, Artificial Sequence
  Synthetic peptide
QIQLVQSGPALKKPGETVKISCKASGYTFTDYSMHWIKQAPGKGLKWMGWISTETGEPTYADGFKGRFDFSLETSADTAYLSINNLTNEDTATYFCTRGLWSSFAYWGQGTLVTVSA

SEQ ID NO: 154 - protein, 111 aa, Artificial Sequence
  Synthetic peptide
DIVLTQSPASLAVSLGQRATISCRASKSVSTSGYSYIHWYQQKPGQPPKLLIYLASNLESGVPARFSGSGSGTDFTLNIHPVEEEDAATYYCQHSRELPLTFGAGTKLELK

SEQ ID NO: 155 - protein, 118 aa, Artificial Sequence
  Synthetic peptide
DVQLVESGGGLVQPRGSRKLSCAASGFTFSSFGMHWVRQAPEKGLEWVAYISSDSRTIYYADTVKGRFTISRDNPTNTLFLQMTSLRSEDTAMYYCARDYGRTYEAYWGQGTLVTVSA

SEQ ID NO: 156 - protein, 107 aa, Artificial Sequence
  Synthetic peptide
DIQMIQSPSSMFASLGDRVSLSCRASQDIGGNLDWYQQKPGGTIKLLIYSTSNLNSGVPSRFSGSGSGSDYSLTITSLESEDFADYYCLQRNAYPLTFGAGTKLELK

SEQ ID NO: 157 - protein, 118 aa, Artificial Sequence
  Synthetic peptide
EVKLMESGGDLVKPGGSLKLSCAASGFTFSSYAMSWVRQTPEKRLEWVASIRSGGTTYYPDSVKGRFTISRDNARNILYLRMSSLRSEDTAIYYCAKVGGNPYPMDYWGQGTSVTVSS

SEQ ID NO: 158 - protein, 108 aa, Artificial Sequence
  Synthetic peptide
EIVLTQSPTTMAASPGEKITITCSASSSISSNYLHWYQQKPGFSPKLLIYRTSNLASGVPARFSGSGSGTSYSLTIGTMEAEDVATYYCQQGSSIPLTFGAGTKLELK

SEQ ID NO: 159 - protein, 122 aa, Artificial Sequence
  Synthetic peptide
QVQLQQSGAELVRPGTSVKVSCKASGYAFSNYLIEWVKQRPGQGLEWIGVINPGSGGTNYNEKFKGKATMTADKSSSTAYMHLSNLTSEDSVVYFCARSYFGRSYPYTMDYWGQGTSVTVSS

SEQ ID NO: 160 - protein, 111 aa, Artificial Sequence
  Synthetic peptide
DIVLTQSPASLAVSLGQRATISCKASQSVDYDGDNYVNWYQQKVGQPPKLLISAASNLESGIPARFSGSGSGTDFTLNIHPVEEEDAATYYCQQSNEDPFTFGSGTKLEIK

SEQ ID NO: 161 - protein, 120 aa, Artificial Sequence
  Synthetic peptide
QVQLQQSGPELVRPGVSVKISCKGSGYTFTDYAMHWVKQSHAKSLEWIGVISTYSGNTNYNQKFQDKATMTVDKSSSTAYMALARLTSDDSAIYYCARRGDYSLYAMDYWGQGTSVTVSS

SEQ ID NO: 162 - protein, 112 aa, Artificial Sequence
  Synthetic peptide
NIMMTQSPSSLAVSAGEKVTMSCKSSQSVLFSSNQKNYLAWYQQKPGQSPRLLIYWASTRESGVPDRFTGSGSGTDFTLTISNVQAEDLAVYYCHQYLSSRTFGAGTKLELK

SEQ ID NO: 163 - protein, 118 aa, Artificial Sequence; identical to SEQ ID NO: 155
  Synthetic peptide

SEQ ID NO: 164 - protein, 111 aa, Artificial Sequence
  Synthetic peptide
DIVLTQSPASLALSLGQRATISCRASESVDNYGISFMNWFQQKPGQPPKLLIYAASNQGSGVPARFSGSGSGTDFSLNIHPMEEDDTAMYFCQQSKEVPLTFGAGTKLELK

SEQ ID NO: 165 - protein, 119 aa, Artificial Sequence
  Synthetic peptide
EVRLVESGGGLMQPGGSLKLPCAASGFPFSSSAMSWVRQTPEKRLEWVASINSDGNTYYPDSVKGRFTISRDSARNILYLQMSSLRSEDTAMYYCTRNGDYRYDEFAYWGQGTLVTVSA

SEQ ID NO: 166 - protein, 108 aa, Artificial Sequence
  Synthetic peptide
QIVLTQSPAIMSASLGERVTMTCTASSSVSSSYLHWYQQKPGSSPKLWIYSTSNLASGVPARFSGSGSGTSYSLTISSMEAEDAATYYCHQYHRSPPTFGAGTKLELK

SEQ ID NO: 167 - protein, 119 aa, Artificial Sequence
  Synthetic peptide
QVQLQQSGAELAKPGASVKMSCKASGYTFTGYWMHWVKQRPGQGLEWLGYINPSTGYTESNQKFKDKATLTADKSSTTAYMQLRSLTPEDSAVYYCAREGITTVLVDYWGQGTTLTVSS

SEQ ID NO: 168 - protein, 112 aa, Artificial Sequence; identical to SEQ ID NO: 162
  Synthetic peptide

SEQ ID NO: 169 - protein, 121 aa, Artificial Sequence
  Synthetic peptide
QVQLKQSGPELEKPGASVKISCKASGYSFTGYNMNWVKQSNGKSLEWIGNIDPYYGGSTYNQKFTGKATLTVDKSSSTAYMQLKSLTSEDSAVYYCARERSGYVFSAMDYWGQGTSVTVSS

SEQ ID NO: 170 - protein, 112 aa, Artificial Sequence; identical to SEQ ID NO: 162
  Synthetic peptide

SEQ ID NO: 171 - protein, 123 aa, Artificial Sequence
  Synthetic peptide
EVQLQQSGPELVKPGGSMKISCKASGYSFTGYTMNWVKRSHGKNLEWIGLINPYNGVTTYNQNFKGKATLAVDKSSSTAYMELLGLTSEDSAVYYCTRDPLYYGYRDSTMDYWGQGTSVTVSS

SEQ ID NO: 172 - protein, 112 aa, Artificial Sequence; identical to SEQ ID NO: 140
  Synthetic peptide

SEQ ID NO: 173 - protein, 117 aa, Artificial Sequence
  Synthetic peptide
EVQLQQSGAELARPGASVKMSCKASGYTFTSYTMHWIKQRPGQGQEWIGYINPSSTYTHYIKKFKDKATLTADKSSSTAYMQLRSLTSEDSAVYYCSRGELGGFAYWGQGTLVTVSA

SEQ ID NO: 174 - protein, 107 aa, Artificial Sequence
  Synthetic peptide
DIQMIQSPSSMFASLGDRVSLSCRASQGIRGNLDWYQQKPGGTIKLLIYSTSILNSGVPSRFSGSGSGSDYSLTITSLESEDFADYYCLQRNAYPLTFGSGTKLELK

SEQ ID NO: 175 - protein, 119 aa, Artificial Sequence
  Synthetic peptide
EVKLVESGGGLMKPGGSLKLSCAASGFTFSSFALSWVRQTPEKRLEWVASIRSGGITYHADSVKGRFTISRDNAGNILYLQMNSLRSEDTAMYFCARVSTATYYGMDYWGQGTSVTVSS

SEQ ID NO: 176 - protein, 219 aa, Mus musculus
  ref <308>: NCBI / NP_061247.1
  ref <309>: 2017-08-07
  ref <313>: (1)..(219)
MASTGLQILGIVLTLLGWVNALVSCALPMWKVTAFIGNSIVVAQMVWEGLWMSCVVQSTGQMQCKVYDSLLALPQDLQAARALCVVTLLIVLLGLLVYLAGAKCTTCVEDRNSKSRLVLISGIIFVISGVLTLIPVCWTAHSIIQDFYNPLVADAQKRELGASLYLGWAASGLLLLGGGLLCCACSSGGTQGPRHYMACYSTSVPHSRGPSEYPTKNYV

SEQ ID NO: 177 - protein, 80 aa, Artificial Sequence
  Synthetic peptide
MASAGMQILGVVLTLLGWVNGLVSCALPMWKVTAFIGNSIVVAQVVWEGLWMSCVVQSTGQMQCKVYDSLLALPQDLQAA

SEQ ID NO: 178 - protein, 220 aa, Artificial Sequence
  Synthetic peptide
MASAGMQILGVVLTLLGWVNGLVSCALPMWKVTAFIGNSIVVAQVVWEGLWMSCVVQSTGQMQCKVYDSLLALPQDLQAARALCVIALLVALFGLLVYLAGAKCTTCVEEKDSKARLVLTSGIVFVISGVLTLIPVCWTAHAVIRDFYNPLVAEAQKRELGASLYLGWAASGLLLLGGGLLCCTCPSGGSQGPSHYMARYSTSAPAISRGPSEYPTKNYV

SEQ ID NO: 179 - protein, 322 aa, Artificial Sequence
  Synthetic peptide
CAGATCGTGCTGACTCAGAGTCCTTCAATTATGTCCGTGAGCCCAGGCGAGAAGGTCACCATCACATGCAGTGCCTCCAGCTCTGTCTCATACATGCACTGGTTCCAGCAGAAGCCAGGGACCAGTCCCAAGCTGTGCATCTACTCTACATCGAACCTGGCCTCCGGAGTGCCCGCAAGGTTTAGCGGTCGGGGCTCTGGAACTTCATACTCCCTGACCATCTCGCGGGTGGCCGCTGAGGATGCAGCAACATACTATTGCCAGCAGAGGTCCAATTATCCCCCTTGGACATTCGGCGGAGGTACCAAACTCGAGATTAAGC

SEQ ID NO: 180 - protein, 351 aa, Artificial Sequence
  Synthetic peptide
GAAGTCCAGCTGCAGCAGTCTGGCCCTGAACTGGTGAAGCCTGGCGCCAGCATGAAGATCTCCTGCAAGGCCAGCGGCTACTCCTTCACCGGCTATACAATGAACTGGGTGAAGCAGTCCCACGGCAAGAATCTGGAGTGGATCGGCCTGATCAACCCATACAATGGCGGCACCATCTACAACCAGAAGTTTAAGGGCAAGGCCACCCTGACAGTGGACAAGAGCTCCTCTACCGCCTACATGGAGCTGCTGTCTCTGACAAGCGAGGACTCCGCCGTGTACTATTGCGCCCGGGACTACGGCTTCGTGCTGGACTATTGGGGCCAGGGCACCACACTGACAGTGAGCTCC

SEQ ID NO: 181 - protein, 107 aa, Artificial Sequence
  Synthetic peptide
QIVLTQSPSIMSVSPGEKVTITCSASSSVSYMHWFQQKPGTSPKLCIYSTSNLASGVPARFSGRGSGTSYSLTISRVAAEDAATYYCQQRSNYPPWTFGGGTKLEIK

SEQ ID NO: 182 - protein, 117 aa, Artificial Sequence
  Synthetic peptide
EVQLQQSGPELVKPGASMKISCKASGYSFTGYTMNWVKQSHGKNLEWIGLINPYNGGTIYNQKFKGKATLTVDKSSSTAYMELLSLTSEDSAVYYCARDYGFVLDYWGQGTTLTVSS

SEQ ID NO: 183 - DNA, 324 bp, Artificial Sequence
  Synthetic polynucleotide
gaaattgtgctcacccagtctccagcactcatggctgcatctccaggggagaaggtcaccatcacctgcagtgtcagctcaagtataagttccagcaacttgcactggtaccagcagaagtcaggaacctcccccaaactctggatttatggcacatccaacctggcttctggagtccctgttcgcttcagtggcagtggatctgggacctcttattctctcacaatcagcaacatggaggctgaagatgctgccacttattactgtcaacagtggagtagttacccacacacgttcggaggggggaccaagctggaaataaaa

SEQ ID NO: 184 - DNA, 378 bp, Artificial Sequence
  Synthetic polynucleotide
caggtccaaatgcagcagtctggagctgagctggtaaggcctgggacttcagtgaaggtgtcctgcaaggcttctggatacgccttcactaattacttgatagagtgggtaaagcagaggcctggacagggccttgagtggattggactgattaatcctggaagtggtggtactaattacaatgagaagttcaagggcaaggcaacactgactgcagacaaatcctccaccactgcctacatgcagctcagcagcctgacatctgatgactctgcggtttatttctgtgcaagacggtcccctctagggagttggatctactatgcttacgacggtgttgcttactggggccaagggactctggtcactgtctctgca

SEQ ID NO: 185 - protein, 108 aa, Artificial Sequence
  Synthetic peptide
EIVLTQSPALMAASPGEKVTITCSVSSSISSSNLHWYQQKSGTSPKLWIYGTSNLASGVPVRFSGSGSGTSYSLTISNMEAEDAATYYCQQWSSYPHTFGGGTKLEIK

SEQ ID NO: 186 - protein, 126 aa, Artificial Sequence
  Synthetic peptide
QVQMQQSGAELVRPGTSVKVSCKASGYAFTNYLIEWVKQRPGQGLEWIGLINPGSGGTNYNEKFKGKATLTADKSSTTAYMQLSSLTSDDSAVYFCARRSPLGSWIYYAYDGVAYWGQGTLVTVSA

SEQ ID NO: 187 - DNA, 645 bp, Mus musculus
gatattgtgctaactcagtctccagccaccctgtctgtgactccaggaaatagcgtcagtctttcctgcagggccagccaaagtattggcggtaacctacactggtatcaacaaaaatcacatgagtctccaaggcttctcatcaagtatgcttcccagtccatctctgggatcccctccaggttcagtggcagtggatcagggacagatttcactctcagtatcaacagtgtggagactgaagattttggaatgtatttctgtcaacagagtaacagctggccttacacgttcggaggggggaccaagctggaaataaaacgggcagatgctgcaccaactgtatccatcttcccaccatccagtgagcagttaacatctggaggtgcctcagtcgtgtgcttcttgaacaacttctaccccaaagacatcaatgtcaagtggaagattgatggcagtgaacgacaaaatggcgtcctgaacagttggactgatcaggacagcaaagacagcacctacagcatgagcagcaccctcacgttgaccaaggacgagtatgaacgacataacagctatacctgtgaggccactcacaagacatcaacttcacccattgtcaagagcttcaacaggaatgagtgttag

SEQ ID NO: 188 - DNA, 1335 bp, Mus musculus
gacgtgcagcttcaggagtcaggacctagcctcgtgaaaccttctcagactctgtccctcacctgttctgtcactggcgactccatcaccagtgattactggagctggatccggaaattcccagggaatagacttgagtacatggggtacgtaagctacagtggtagcacttactacaatccatctctcaaaagtcgaatctccatcacccgagacacatccaagaaccagtactacctggatttgaattctgtgactactgaggacacagccacatattactgtgcaaactgggacggtgattactggggccaagggactctggtcactgtctcttcagcagctaaaacaacagccccatcggtctatccactggcccctgtgtgtggagatacaactggctcctcggtgactctaggatgcctggtcaagggttatttccctgagccagtgaccttgacctggaactctggatccctgtccagtggtgtgcacaccttcccagctgtcctgcagtctgacctctacaccctcagcagctcagtgactgtaacctcgagcacctggcccagccagtccatcacctgcaatgtggcccacccggcaagcagcaccaaggtggacaagaaaattgagcccagagggcccacaatcaagccctgtcctccatgcaaatgcccagcacctaacctcttgggtggaccatccgtcttcatcttccctccaaagatcaaggatgtactcatgatctccctgagccccatagtcacatgtgtggtggtggatgtgagcgaggatgacccagatgtccagatcagctggtttgtgaacaacgtggaagtacacacagctcagacacaaacccatagagaggattacaacagtactctccgggtggtcagtgccctccccatccagcaccaggactggatgagtggcaaggagttcaaatgcaaggtcaacaacaaagacctcccagcgcccatcgagagaaccatctcaaaacccaaagggtcagtaagagctccacaggtatatgtcttgcctccaccagaagaagagatgactaagaaacaggtcactctgacctgcatggtcacagacttcatgcctgaagacatttacgtggagtggaccaacaacgggaaaacagagctaaactacaagaacactgaaccagtcctggactctgatggttcttacttcatgtacagcaagctgagagtggaaaagaagaactgggtggaaagaaatagctactcctgttcagtggtccacgagggtctgcacaatcaccacacgactaagagcttctcccggactccgggtaaatga

SEQ ID NO: 189 - DNA, 8806 bp, Artificial Sequence
  Synthetic peptide
aatgtagtcttatgcaatactcttgtagtcttgcaacatggtaacgatgagttagcaacatgccttacaaggagagaaaaagcaccgtgcatgccgattggtggaagtaaggtggtacgatcgtgccttattaggaaggcaacagacgggtctgacatggattggacgaaccactgaattgccgcattgcagagatattgtatttaagtgcctagctcgatacataaacgggtctctctggttagaccagatctgagcctgggagctctctggctaactagggaacccactgcttaagcctcaataaagcttgccttgagtgcttcaagtagtgtgtgcccgtctgttgtgtgactctggtaactagagatccctcagacccttttagtcagtgtggaaaatctctagcagtggcgcccgaacagggacttgaaagcgaaagggaaaccagaggagctctctcgacgcaggactcggcttgctgaagcgcgcacggcaagaggcgaggggcggcgactggtgagtacgccaaaaattttgactagcggaggctagaaggagagagatgggtgcgagagcgtcagtattaagcgggggagaattagatcgcgatgggaaaaaattcggttaaggccagggggaaagaaaaaatataaattaaaacatatagtatgggcaagcagggagctagaacgattcgcagttaatcctggcctgttagaaacatcagaaggctgtagacaaatactgggacagctacaaccatcccttcagacaggatcagaagaacttagatcattatataatacagtagcaaccctctattgtgtgcatcaaaggatagagataaaagacaccaaggaagctttagacaagatagaggaagagcaaaacaaaagtaagaccaccgcacagcaagcggccgctgatcttcagacctggaggaggagatatgagggacaattggagaagtgaattatataaatataaagtagtaaaaattgaaccattaggagtagcacccaccaaggcaaagagaagagtggtgcagagagaaaaaagagcagtgggaataggagctttgttccttgggttcttgggagcagcaggaagcactatgggcgcagcgtcaatgacgctgacggtacaggccagacaattattgtctggtatagtgcagcagcagaacaatttgctgagggctattgaggcgcaacagcatctgttgcaactcacagtctggggcatcaagcagctccaggcaagaatcctggctgtggaaagatacctaaaggatcaacagctcctggggatttggggttgctctggaaaactcatttgcaccactgctgtgccttggaatgctagttggagtaataaatctctggaacagatttggaatcacacgacctggatggagtgggacagagaaattaacaattacacaagcttaatacactccttaattgaagaatcgcaaaaccagcaagaaaagaatgaacaagaattattggaattagataaatgggcaagtttgtggaattggtttaacataacaaattggctgtggtatataaaattattcataatgatagtaggaggcttggtaggtttaagaatagtttttgctgtactttctatagtgaatagagttaggcagggatattcaccattatcgtttcagacccacctcccaaccccgaggggacccgacaggcccgaaggaatagaagaagaaggtggagagagagacagagacagatccattcgattagtgaacggatctcgacggtatcggttaacttttaaaagaaaaggggggattggggggtacagtgcaggggaaagaatagtagacataatagcaacagacatacaaactaaagaattacaaaaacaaattacaaaaattcaaaattttccgataagcttgggagttccgcgttacataacttacggtaaatggcccgcctggctgaccgcccaacgacccccgcccattgacgtcaataatgacgtatgttcccatagtaacgccaatagggactttccattgacgtcaatgggtggagtatttacggtaaactgcccacttggcagtacatcaagtgtatcatatgccaagtacgccccctattgacgtcaatgacggtaaatggcccgcctggcattatgcccagtacatgaccttatgggactttcctacttggcagtacatctacgtattagtcatcgctattaccatggtgatgcggttttggcagtacatcaatgggcgtggatagcggtttgactcacggggatttccaagtctccaccccattgacgtcaatgggagtttgttttggcaccaaaatcaacgggactttccaaaatgtcgtaacaactccgccccattgacgcaaatgggcggtaggcgtgtacggtgggaggtctatataagcagagctcgtttagtgaaccgtcagatcgcctggagacgccatccacgctgttttgacctccatagaagacaccgactctagaactagtggatcccccgggctgcaggaattcgtcgactggatccggtaccgaggagatctgccgccgcgatcgccggcgcgccagatctcaagcttaactagttagcggaccgacgcgtacgcggccgctcgagatgagcgggggcgaggagctgttcgccggcatcgtgcccgtgctgatcgagctggacggcgacgtgcacggccacaagttcagcgtgcgcggcgagggcgagggcgacgccgactacggcaagctggagatcaagttcatctgcaccaccggcaagctgcccgtgccctggcccaccctggtgaccaccctctgctacggcatccagtgcttcgcccgctaccccgagcacatgaagatgaacgacttcttcaagagcgccatgcccgagggctacatccaggagcgcaccatccagttccaggacgacggcaagtacaagacccgcggcgaggtgaagttcgagggcgacaccctggtgaaccgcatcgagctgaagggcaaggacttcaaggaggacggcaacatcctgggccacaagctggagtacagcttcaacagccacaacgtgtacatccgccccgacaaggccaacaacggcctggaggctaacttcaagacccgccacaacatcgagggcggcggcgtgcagctggccgaccactaccagaccaacgtgcccctgggcgacggccccgtgctgatccccatcaaccactacctgagcactcagaccaagatcagcaaggaccgcaacgaggcccgcgaccacatggtgctcctggagtccttcagcgcctgctgccacacccacggcatggacgagctgtacaggtccggactcagataagtttaaacccgatatcatcatctagggcggccaattccgcccctctccccccccctaacgttactggccgaagccgcttggaataaggccggtgtgcgtttgtctatatgttattttccaccatattgccgtcttttggcaatgtgagggcccggaaacctggccctgtcttcttgacgagcattcctaggggtctttcccctctcgccaaaggaatgcaaggtctgttgaatgtcgtgaaggaagcagttcctctggaagcttcttgaagacaaacaacgtctgtagcgaccctttgcaggcagcggaaccccccacctggcgacaggtgcctctgcggccaaaagccacgtgtataagatacacctgcaaaggcggcacaaccccagtgccacgttgtgagttggatagttgtggaaagagtcaaatggctctcctcaagcgtattcaacaaggggctgaaggatgcccagaaggtaccccattgtatgggatctgatctggggcctcggtgcacatgctttacatgtgtttagtcgaggttaaaaaaacgtctaggccccccgaaccacggggacgtggttttcctttgaaaaacacgatgataagcttgccacaacccacaaggagacgaccttccatgaccgagtacaagcccacggtgcgcctcgccacccgcgacgacgtcccccgggccgtacgcaccctcgccgccgcgttcgccgactaccccgccacgcgccacaccgtcgacccggaccgccacatcgagcgggtcaccgagctgcaagaactcttcctcacgcgcgtcgggctcgacatcggcaaggtgtgggtcgcggacgacggcgccgcggtggcggtctggaccacgccggagagcgtcgaagcgggggcggtgttcgccgagatcggcccgcgcatggccgagttgagcggttcccggctggccgcgcagcaacagatggaaggcctcctggcgccgcaccggcccaaggagcccgcgtggttcctggccaccgtcggcgtctcgcccgaccaccagggcaagggtctgggcagcgccgtcgtgctccccggagtggaggcggccgagcgcgccggggtgcccgccttcctggagacctccgcgccccgcaacctccccttctacgagcggctcggcttcaccgtcaccgccgacgtcgaggtgcccgaaggaccgcgcacctggtgcatgacccgcaagcccggtgcctgaaattagatcgataccgtcgacaatcaacctctggattacaaaatttgtgaaagattgactggtattcttaactatgttgctccttttacgctatgtggatacgctgctttaatgcctttgtatcatgctattgcttcccgtatggctttcattttctcctccttgtataaatcctggttgctgtctctttatgaggagttgtggcccgttgtcaggcaacgtggcgtggtgtgcactgtgtttgctgacgcaacccccactggttggggcattgccaccacctgtcagctcctttccgggactttcgctttccccctccctattgccacggcggaactcatcgccgcctgccttgcccgctgctggacaggggctcggctgttgggcactgacaattccgtggtgttgtcggggaagctgacgtcctttccatggctgctcgcctgtgttgccacctggattctgcgcgggacgtccttctgctacgtcccttcggccctcaatccagcggaccttccttcccgcggcctgctgccggctctgcggcctcttccgcgtcttcgccttcgccctcagacgagtcggatctccctttgggccgcctccccgcctgaatacgagctcggtacctttaagaccaatgacttacaaggcagctgtagatcttagccactttttaaaagaaaaggggggactggaagggctaattcactcccaacgaagacaagatctgctttttgcttgtactgggtctctctggttagaccagatctgagcctgggagctctctggctaactagggaacccactgcttaagcctcaataaagcttgccttgagtgcttcaagtagtgtgtgcccgtctgttgtgtgactctggtaactagagatccctcagacccttttagtcagtgtggaaaatctctagcagtagtagttcatgtcatcttattattcagtatttataacttgcaaagaaatgaatatcagagagtgagaggaacttgtttattgcagcttataatggttacaaataaagcaatagcatcacaaatttcacaaataaagcatttttttcactgcattctagttgtggtttgtccaaactcatcaatgtatcttatcatgtctggctctagctatcccgcccctaactccgcccatcccgcccctaactccgcccagttccgcccattctccgccccatggctgactaattttttttatttatgcagaggccgaggccgcctcggcctctgagctattccagaagtagtgaggaggcttttttggaggcctagggacgtacccaattcgccctatagtgagtcgtattacgcgcgctcactggccgtcgttttacaacgtcgtgactgggaaaaccctggcgttacccaacttaatcgccttgcagcacatccccctttcgccagctggcgtaatagcgaagaggcccgcaccgatcgcccttcccaacagttgcgcagcctgaatggcgaatgggacgcgccctgtagcggcgcattaagcgcggcgggtgtggtggttacgcgcagcgtgaccgctacacttgccagcgccctagcgcccgctcctttcgctttcttcccttcctttctcgccacgttcgccggctttccccgtcaagctctaaatcgggggctccctttagggttccgatttagtgctttacggcacctcgaccccaaaaaacttgattagggtgatggttcacgtagtgggccatcgccctgatagacggtttttcgccctttgacgttggagtccacgttctttaatagtggactcttgttccaaactggaacaacactcaaccctatctcggtctattcttttgatttataagggattttgccgatttcggcctattggttaaaaaatgagctgatttaacaaaaatttaacgcgaattttaacaaaatattaacgtttacaatttcccaggtggcacttttcggggaaatgtgcgcggaacccctatttgtttatttttctaaatacattcaaatatgtatccgctcatgagacaataaccctgataaatgcttcaataatattgaaaaaggaagagtatgagtattcaacatttccgtgtcgcccttattcccttttttgcggcattttgccttcctgtttttgctcacccagaaacgctggtgaaagtaaaagatgctgaagatcagttgggtgcacgagtgggttacatcgaactggatctcaacagcggtaagatccttgagagttttcgccccgaagaacgttttccaatgatgagcacttttaaagttctgctatgtggcgcggtattatcccgtattgacgccgggcaagagcaactcggtcgccgcatacactattctcagaatgacttggttgagtactcaccagtcacagaaaagcatcttacggatggcatgacagtaagagaattatgcagtgctgccataaccatgagtgataacactgcggccaacttacttctgacaacgatcggaggaccgaaggagctaaccgcttttttgcacaacatgggggatcatgtaactcgccttgatcgttgggaaccggagctgaatgaagccataccaaacgacgagcgtgacaccacgatgcctgtagcaatggcaacaacgttgcgcaaactattaactggcgaactacttactctagcttcccggcaacaattaatagactggatggaggcggataaagttgcaggaccacttctgcgctcggcccttccggctggctggtttattgctgataaatctggagccggtgagcgtgggtctcgcggtatcattgcagcactggggccagatggtaagccctcccgtatcgtagttatctacacgacggggagtcaggcaactatggatgaacgaaatagacagatcgctgagataggtgcctcactgattaagcattggtaactgtcagaccaagtttactcatatatactttagattgatttaaaacttcatttttaatttaaaaggatctaggtgaagatcctttttgataatctcatgaccaaaatcccttaacgtgagttttcgttccactgagcgtcagaccccgtagaaaagatcaaaggatcttcttgagatcctttttttctgcgcgtaatctgctgcttgcaaacaaaaaaaccaccgctaccagcggtggtttgtttgccggatcaagagctaccaactctttttccgaaggtaactggcttcagcagagcgcagataccaaatactgtccttctagtgtagccgtagttaggccaccacttcaagaactctgtagcaccgcctacatacctcgctctgctaatcctgttaccagtggctgctgccagtggcgataagtcgtgtcttaccgggttggactcaagacgatagttaccggataaggcgcagcggtcgggctgaacggggggttcgtgcacacagcccagcttggagcgaacgacctacaccgaactgagatacctacagcgtgagctatgagaaagcgccacgcttcccgaagggagaaaggcggacaggtatccggtaagcggcagggtcggaacaggagagcgcacgagggagcttccagggggaaacgcctggtatctttatagtcctgtcgggtttcgccacctctgacttgagcgtcgatttttgtgatgctcgtcaggggggcggagcctatggaaaaacgccagcaacgcggcctttttacggttcctggccttttgctggccttttgctcacatgttctttcctgcgttatcccctgattctgtggataaccgtattaccgcctttgagtgagctgataccgctcgccgcagccgaacgaccgagcgcagcgagtcagtgagcgaggaagcggaagagcgcccaatacgcaaaccgcctctccccgcgcgttggccgattcattaatgcagctggcacgacaggtttcccgactggaaagcgggcagtgagcgcaacgcaattaatgtgagttagctcactcattaggcaccccaggctttacactttatgcttccggctcgtatgttgtgtggaattgtgagcggataacaatttcacacaggaaacagctatgaccatgattacgccaagcgcgcaattaaccctcactaaagggaacaaaagctggagctgcaagctt

SEQ ID NO: 190 - protein, 220 aa, Artificial Sequence
  Synthetic peptide
  misc_feature (143)..(143): Xaa can be any naturally occurring amino acid
MASAGMQILGVVLTLLGWVNGLVSCALPMWKVTAFIGNSIVVAQVVWEGLWMSCVVQSTGQMQCKVYDSLLALPQDLQAARALCVIALLVALFGLLVYLAGAKCTTCVEEKDSKARLVLTSGIVFVISGVLTLIPVCWTAHAXIRDFYNPLVAEAQKRELGASLYLGWAASGLLLLGGGLLCCTCPSGGSQGPSHYMARYSTSAPAISRGPSEYPTKNYV

SEQ ID NO: 191 - DNA, 68 bp, Artificial Sequence
  Synthetic polynucleotide
cagaaactcatctcagaagaggatctggcagcaaatgatatcctggattacaaggatgacgacgataa

SEQ ID NO: 192 - DNA, 683 bp, Homo sapiens
  ref <308>: NCBI / NM_021195.4
  ref <309>: 2017-06-04
  ref <313>: (1)..(683)
ccgcgatcgccatggcctctgccggaatgcagatcctgggagtcgtcctgacactgctgggctgggtgaatggcctggtctcctgtgccctgcccatgtggaaggtgaccgctttcatcggcaacagcatcgtggtggcccaggtggtgtgggagggcctgtggatgtcctgcgtggtgcagagcaccggccagatgcagtgcaaggtgtacgactcactgctggcgctgccacaggacctgcaggctgcacgtgccctctgtgtcatcgccctccttgtggccctgttcggcttgctggtctaccttgctggggccaagtgtaccacctgtgtggaggagaaggattccaaggcccgcctggtgctcacctctgggattgtctttgtcatctcaggggtcctgacgctaatccccgtgtgctggacggcgcatgccgtcatccgggacttctataaccccctggtggctgaggcccaaaagcgggagctgggggcctccctctacttgggctgggcggcctcaggccttttgttgctgggtggggggttgctgtgctgcacttgcccctcgggggggtcccagggccccagccattacatggcccgctactcaacatctgcccctgccatctctcgggggccctctgagtaccctaccaagaattacgtcacgcgtacgcgg

SEQ ID NO: 193 - DNA, 677 bp, Mus musculas
  ref <308>: NCBI / NM_018777.4
  ref <309>: 2017-08-07
  ref <313>: (1)..(677)
gccgcgatcgccatggcctctactggtctgcaaatcttggggatcgtcctgaccctgcttggctgggtcaacgccctggtgtcctgtgccctgcccatgtggaaggtgaccgccttcatcggcaacagcatcgtcgtggcccagatggtgtgggaggggctgtggatgtcctgtgtggttcagagcactggccagatgcagtgcaaggtgtatgactcactgttggcgctgccccaggacctgcaggctgccagagccctctgtgttgtcaccctcctcattgtcctgcttggcctgctcgtgtacctggctggagccaagtgcactacctgtgtggaagataggaactccaagtctcgtctggtgctcatctctggcatcatctttgtcatttctggggtcctgacgctcattcctgtctgctggactgcccactctatcatccaggacttctacaaccccttggtggctgatgctcaaaagcgggagctgggggcctccctctacctgggctgggcagcctcaggccttttgctgctgggtggagggctactatgctgcgcctgctcttctggagggacccagggacccagacattacatggcctgctattctacatctgtcccacattctcggggaccctccgaatatcccaccaagaattatgtgacgcgtac

SEQ ID NO: 194 - DNA, 683 bp, Artificial Sequence
  Synthetic polynucleotide
cgcgatcgccatggcctctgccggaatgcagatcctgggagtcgtcctgacactgctgggctgggtgaatggcctggtctcctgtgccctgcccatgtggaaggtgaccgctttcatcggcaacagcatcgtggtggcccaggtggtgtgggagggcctgtggatgtcctgcgtggtgcagagcaccggccagatgcagtgcaaggtgtacgactcactgctggcgctgccacaggacctgcaggctgcacgtgccctctgtgtcatcgccctccttgtggccctgttcggcttgctggtctaccttgctggggccaagtgtaccacctgtgtggaggagaaggattccaaggcccgcctggtgctcacctctgggattgtctttgtcatctcaggggtcctgacgctaatccccgtgtgctggacggcgcatgccatcatccgggacttctataaccccctggtggctgaggcccaaaagcgggagctgggggcctccctctacttgggctgggcggcctcaggccttttgttgctgggtggggggttgctgtgctgcacttgcccctcgggggggtcccagggccccagccattacatggcccgctactcaacatctgcccctgccatctctcgggggccctctgagtaccctaccaagaattacgtcacgcgtacgcggc

SEQ ID NO: 195 - DNA, 672 bp, Homo sapiens
  ref <308>: NCBI / NM_020982.3
  ref <309>: 2017-04-15
  ref <313>: (1)..(672)
gccgcgatcgccatggcttcgaccggcttagaactgctgggcatgaccctggctgtgctgggctggctggggaccctggtgtcctgcgccctgcccctgtggaaggtgaccgccttcatcggcaacagcatcgtggtggcccaggtggtgtgggagggcctgtggatgtcctgcgtggtgcagagcacgggccagatgcagtgcaaggtgtacgactcactgctggctctgccgcaggacctgcaggccgcacgtgccctctgtgtcattgccctcctgctggccctgcttggcctcctggtggccatcacaggtgcccagtgtaccacgtgtgtggaggacgaaggtgccaaggcccgtatcgtgctcaccgcgggggtcatcctcctcctcgccggcatcctggtgctcatccctgtgtgctggacggcgcacgccatcatccaggacttctacaaccccctggtggctgaggccctcaagcgggagctgggggcctccctctacctgggctgggcggcggctgcactgcttatgctgggcggggggctcctctgctgcacgtgccccccgccccaggtcgagcggccccgcggacctcggctgggctactccatcccctcccgctcgggtgcatctggactggacaagagggactacgtgacgcgtacg

SEQ ID NO: 196 - DNA, 651 bp, Homo sapiens
  ref <308>: NCBI / NM_001305.4
  ref <309>: 2017-07-10
  ref <313>: (1)..(651)
ccgcgatcgccatggcctccatggggctacaggtaatgggcatcgcgctggccgtcctgggctggctggccgtcatgctgtgctgcgcgctgcccatgtggcgcgtgacggccttcatcggcagcaacattgtcacctcgcagaccatctgggagggcctatggatgaactgcgtggtgcagagcaccggccagatgcagtgcaaggtgtacgactcgctgctggcactgccgcaggacctgcaggcggcccgcgccctcgtcatcatcagcatcatcgtggctgctctgggcgtgctgctgtccgtggtggggggcaagtgtaccaactgcctggaggatgaaagcgccaaggccaagaccatgatcgtggcgggcgtggtgttcctgttggccggccttatggtgatagtgccggtgtcctggacggcccacaacatcatccaagacttctacaatccgctggtggcctccgggcagaagcgggagatgggtgcctcgctctacgtcggctgggccgcctccggcctgctgctccttggcggggggctgctttgctgcaactgtccaccccgcacagacaagccttactccgccaagtattctgctgcccgctctgctgctgccagcaactacgtgacgcgtacgcggc

SEQ ID NO: 197 - DNA, 680 bp, Homo sapiens
  ref <308>: NCBI / NM_001306.3
  ref <309>: 2017-07-10
  ref <313>: (1)..(680)
gccgcgatcgccatgtccatgggcctggagatcacgggcaccgcgctggccgtgctgggctggctgggcaccatcgtgtgctgcgcgttgcccatgtggcgcgtgtcggccttcatcggcagcaacatcatcacgtcgcagaacatctgggagggcctgtggatgaactgcgtggtgcagagcaccggccagatgcagtgcaaggtgtacgactcgctgctggcactgccacaggaccttcaggcggcccgcgccctcatcgtggtggccatcctgctggccgccttcgggctgctagtggcgctggtgggcgcccagtgcaccaactgcgtgcaggacgacacggccaaggccaagatcaccatcgtggcaggcgtgctgttccttctcgccgccctgctcaccctcgtgccggtgtcctggtcggccaacaccattatccgggacttctacaaccccgtggtgcccgaggcgcagaagcgcgagatgggcgcgggcctgtacgtgggctgggcggccgcggcgctgcagctgctggggggcgcgctgctctgctgctcgtgtcccccacgcgagaagaagtacacggccaccaaggtcgtctactccgcgccgcgctccaccggcccgggagccagcctgggcacaggctacgaccgcaaggactacgtcacgcgtac

SEQ ID NO: 198 - protein, 214 aa, Artificial Sequence
  Synthetic peptide
DIVLTQSPATLSVTPGNSVSLSCRASQSIGGNLHWYQQKSHESPRLLIKYASQSISGIPSRFSGSGSGTDFTLSINSVETEDFGMYFCQQSNSWPYTFGGGTKLEIKRADAAPTVSIFPPSSEQLTSGGASVVCFLNNFYPKDINVKWKIDGSERQNGVLNSWTDQDSKDSTYSMSSTLTLTKDEYERHNSYTCEATHKTSTSPIVKSFNRNEC

SEQ ID NO: 199 - protein, 444 aa, Artificial Sequence
  Synthetic peptide
DVQLQESGPSLVKPSQTLSLTCSVTGDSITSDYWSWIRKFPGNRLEYMGYVSYSGSTYYNPSLKSRISITRDTSKNQYYLDLNSVTTEDTATYYCANWDGDYWGQGTLVTVSSAAKTTAPSVYPLAPVCGDTTGSSVTLGCLVKGYFPEPVTLTWNSGSLSSGVHTFPAVLQSDLYTLSSSVTVTSSTWPSQSITCNVAHPASSTKVDKKIEPRGPTIKPCPPCKCPAPNLLGGPSVFIFPPKIKDVLMISLSPIVTCVVVDVSEDDPDVQISWFVNNVEVHTAQTQTHREDYNSTLRVVSALPIQHQDWMSGKEFKCKVNNKDLPAPIERTISKPKGSVRAPQVYVLPPPEEEMTKKQVTLTCMVTDFMPEDIYVEWTNNGKTELNYKNTEPVLDSDGSYFMYSKLRVEKKNWVERNSYSCSVVHEGLHNHHTTKSFSRTPGK

SEQ ID NO: 200 - protein, 220 aa, Artificial Sequence; identical to SEQ ID NO: 190
  Synthetic peptide
  misc_feature (143)..(143): Xaa can be any naturally occurring amino acid

SEQ ID NO: 201 - protein, 220 aa, Artificial Sequence; identical to SEQ ID NO: 190
  Synthetic peptide
  misc_feature (143)..(143): Xaa can be any naturally occurring amino acid

SEQ ID NO: 202-207 - skipped (6 entries)

SEQ ID NO: 208 - DNA, 21 bp, Artificial Sequence
  Synthetic polynucleotide
tccagtgtaagttccacttac

SEQ ID NO: 209 - DNA, 9 bp, Artificial Sequence
  Synthetic polynucleotide
agcacatcc

SEQ ID NO: 210 - DNA, 27 bp, Artificial Sequence
  Synthetic polynucleotide
caccagtatcatcgttccccgctcacg

SEQ ID NO: 211 - DNA, 24 bp, Artificial Sequence
  Synthetic polynucleotide
ggctacacctttactacctacacg

SEQ ID NO: 212 - DNA, 24 bp, Artificial Sequence
  Synthetic polynucleotide
attaatcctagcagtggatatact

SEQ ID NO: 213 - DNA, 27 bp, Artificial Sequence
  Synthetic polynucleotide
gcaaacggggattactacgtcgcttac

SEQ ID NO: 214 - DNA, 18 bp, Artificial Sequence
  Synthetic polynucleotide
gagaatatttacagttat

SEQ ID NO: 215 - DNA, 9 bp, Artificial Sequence
  Synthetic polynucleotide
aatgcaaaa

SEQ ID NO: 216 - DNA, 27 bp, Artificial Sequence
  Synthetic polynucleotide
caacatcattatactgttccgtggacg

SEQ ID NO: 217 - DNA, 24 bp, Artificial Sequence
  Synthetic polynucleotide
ggtttcactttcagtgattactgg

SEQ ID NO: 218 - DNA, 30 bp, Artificial Sequence
  Synthetic polynucleotide
attagattgaaatctgataattatgcaaca

SEQ ID NO: 219 - DNA, 24 bp, Artificial Sequence
  Synthetic polynucleotide
aatgatggccccccctcggggtgt

SEQ ID NO: 220 - DNA, 18 bp, Artificial Sequence
  Synthetic polynucleotide
gagaatatttacagttat

SEQ ID NO: 221 - DNA, 9 bp, Artificial Sequence
  Synthetic polynucleotide
aatgcaaaa

SEQ ID NO: 222 - DNA, 27 bp, Artificial Sequence
  Synthetic polynucleotide
caacatcattatactgttccgtggacg

SEQ ID NO: 223 - DNA, 24 bp, Artificial Sequence
  Synthetic polynucleotide
ggattcactttcagtaattactgg

SEQ ID NO: 224 - DNA, 30 bp, Artificial Sequence; identical to SEQ ID NO: 218
  Synthetic polynucleotide

SEQ ID NO: 225 - DNA, 24 bp, Artificial Sequence
  Synthetic polynucleotide
aatgatggccccccctcggggtgt

SEQ ID NO: 226 - DNA, 33 bp, Artificial Sequence
  Synthetic polynucleotide
cagagccttgtacacagtgatggaaacacctat

SEQ ID NO: 227 - DNA, 9 bp, Artificial Sequence
  Synthetic polynucleotide
aaagtttcc

SEQ ID NO: 228 - DNA, 27 bp, Artificial Sequence
  Synthetic polynucleotide
tctcaaagtacacatgttccttacacg

SEQ ID NO: 229 - DNA, 24 bp, Artificial Sequence
  Synthetic polynucleotide
ggctacacctttactagctacacg

SEQ ID NO: 230 - DNA, 24 bp, Artificial Sequence
  Synthetic polynucleotide
attaatcctagcagtacttatact

SEQ ID NO: 231 - DNA, 30 bp, Artificial Sequence
  Synthetic polynucleotide
tcaagaggggaactgggagggtttgcttac

SEQ ID NO: 232 - DNA, 33 bp, Artificial Sequence
  Synthetic polynucleotide
cagagcattgtacatagtaatggaaacacctat

SEQ ID NO: 233 - DNA, 9 bp, Artificial Sequence
  Synthetic polynucleotide
aaagtttcc

SEQ ID NO: 234 - DNA, 27 bp, Artificial Sequence
  Synthetic polynucleotide
tttcaaggttcacatgttccattcacg

SEQ ID NO: 235 - DNA, 24 bp, Artificial Sequence
  Synthetic polynucleotide
ggatacatattcactcactatatt

SEQ ID NO: 236 - DNA, 24 bp, Artificial Sequence
  Synthetic polynucleotide
attaatccttacaatgatggtact

SEQ ID NO: 237 - DNA, 39 bp, Artificial Sequence
  Synthetic polynucleotide
gcaagatactacggctacccttactattctatggactac

SEQ ID NO: 238 - DNA, 36 bp, Artificial Sequence
  Synthetic polynucleotide
cagagtctgctcaacagtagaacccgaaagaactac

SEQ ID NO: 239 - DNA, 9 bp, Artificial Sequence
  Synthetic polynucleotide
tgggcatcc

SEQ ID NO: 240 - DNA, 24 bp, Artificial Sequence
  Synthetic polynucleotide
aagcaatcttattatctgtacacg

SEQ ID NO: 241 - DNA, 27 bp, Artificial Sequence
  Synthetic polynucleotide
ggctactccatcaccagtggttattac

SEQ ID NO: 242 - DNA, 21 bp, Artificial Sequence
  Synthetic polynucleotide
atcagctacgatggtggcatt

SEQ ID NO: 243 - DNA, 30 bp, Artificial Sequence
  Synthetic polynucleotide
gcaagatttggtaagggggctatggactac

SEQ ID NO: 244 - DNA, 21 bp, Artificial Sequence
  Synthetic polynucleotide
tcaagtgtaagttccagttac

SEQ ID NO: 245 - DNA, 9 bp, Artificial Sequence
  Synthetic polynucleotide
agcacatcc

SEQ ID NO: 246 - DNA, 27 bp, Artificial Sequence
  Synthetic polynucleotide
caccagtatcatcgttccccacccacg

SEQ ID NO: 247 - DNA, 24 bp, Artificial Sequence
  Synthetic polynucleotide
ggttactcattcactggctacacc

SEQ ID NO: 248 - DNA, 24 bp, Artificial Sequence
  Synthetic polynucleotide
attaatccttacaatggtggtact

SEQ ID NO: 249 - DNA, 36 bp, Artificial Sequence
  Synthetic polynucleotide
gcaagaggggtctatgattacgacggatttacttac

SEQ ID NO: 250 - DNA, 33 bp, Artificial Sequence; identical to SEQ ID NO: 226
  Synthetic polynucleotide

SEQ ID NO: 251 - DNA, 9 bp, Artificial Sequence
  Synthetic polynucleotide
aaagtttcc

SEQ ID NO: 252 - DNA, 27 bp, Artificial Sequence
  Synthetic polynucleotide
tctcaaagtacacatgttccttacacg

SEQ ID NO: 253 - DNA, 24 bp, Artificial Sequence
  Synthetic polynucleotide
ggctacacctttactacctacacg

SEQ ID NO: 254 - DNA, 24 bp, Artificial Sequence
  Synthetic polynucleotide
attaatcctcgcagtggttatagt

SEQ ID NO: 255 - DNA, 30 bp, Artificial Sequence; identical to SEQ ID NO: 231
  Synthetic polynucleotide

SEQ ID NO: 256 - DNA, 18 bp, Artificial Sequence
  Synthetic polynucleotide
cagaccattggtacatgg

SEQ ID NO: 257 - DNA, 9 bp, Artificial Sequence
  Synthetic polynucleotide
gctgcagcc

SEQ ID NO: 258 - DNA, 27 bp, Artificial Sequence
  Synthetic polynucleotide
caacaactttacagtattcctcggacg

SEQ ID NO: 259 - DNA, 24 bp, Artificial Sequence
  Synthetic polynucleotide
ggatacagattcactgactacaac

SEQ ID NO: 260 - DNA, 24 bp, Artificial Sequence
  Synthetic polynucleotide
attaaccctaacaatggtggtact

SEQ ID NO: 261 - DNA, 30 bp, Artificial Sequence
  Synthetic polynucleotide
gcaagagattacttgtacttctttgactgc

SEQ ID NO: 262 - DNA, 33 bp, Artificial Sequence
  Synthetic polynucleotide
cagagccttgtacacagtaatggaaacacctat

SEQ ID NO: 263 - DNA, 9 bp, Artificial Sequence
  Synthetic polynucleotide
aaagtttcc

SEQ ID NO: 264 - DNA, 27 bp, Artificial Sequence
  Synthetic polynucleotide
tctcaaattacacatgttccgtacacg

SEQ ID NO: 265 - DNA, 24 bp, Artificial Sequence
  Synthetic polynucleotide
ggttataccttcacagactattca

SEQ ID NO: 266 - DNA, 24 bp, Artificial Sequence
  Synthetic polynucleotide
ataagcactgagactggtgagcca

SEQ ID NO: 267 - DNA, 30 bp, Artificial Sequence
  Synthetic polynucleotide
actagaggtctatggtcctcgtttgcttac

SEQ ID NO: 268 - DNA, 30 bp, Artificial Sequence
  Synthetic polynucleotide
aaaagtgtcagtacatctggctatagttat

SEQ ID NO: 269 - DNA, 9 bp, Artificial Sequence
  Synthetic polynucleotide
cttgcatcc

SEQ ID NO: 270 - DNA, 27 bp, Artificial Sequence
  Synthetic polynucleotide
cagcacagtagggagcttccgctcacg

SEQ ID NO: 271 - DNA, 24 bp, Artificial Sequence
  Synthetic polynucleotide
ggattcactttcagtagctttgga

SEQ ID NO: 272 - DNA, 24 bp, Artificial Sequence
  Synthetic polynucleotide
attagtagtgacagtaggaccatc

SEQ ID NO: 273 - DNA, 33 bp, Artificial Sequence
  Synthetic polynucleotide
gcaagagactacggtagaacctacgaggcttac

SEQ ID NO: 274 - DNA, 18 bp, Artificial Sequence
  Synthetic polynucleotide
caggacattggaggaaat

SEQ ID NO: 275 - DNA, 9 bp, Artificial Sequence
  Synthetic polynucleotide
tccacatcc

SEQ ID NO: 276 - DNA, 27 bp, Artificial Sequence
  Synthetic polynucleotide
ctacagcgtaatgcgtatccgctcact

SEQ ID NO: 277 - DNA, 24 bp, Artificial Sequence
  Synthetic polynucleotide
ggattcactttcagtagttatgcc

SEQ ID NO: 278 - DNA, 21 bp, Artificial Sequence
  Synthetic polynucleotide
attagaagtggtggtaccacc

SEQ ID NO: 279 - DNA, 36 bp, Artificial Sequence
  Synthetic polynucleotide
gcaaaagtgggcggtaacccctatcctatggactac

SEQ ID NO: 280 - DNA, 21 bp, Artificial Sequence
  Synthetic polynucleotide
tcaagtataagttccaattac

SEQ ID NO: 281 - DNA, 9 bp, Artificial Sequence
  Synthetic polynucleotide
aggacatcc

SEQ ID NO: 282 - DNA, 27 bp, Artificial Sequence
  Synthetic polynucleotide
cagcagggtagtagtataccgctcacg

SEQ ID NO: 283 - DNA, 24 bp, Artificial Sequence
  Synthetic polynucleotide
ggatacgccttcagtaattacttg

SEQ ID NO: 284 - DNA, 24 bp, Artificial Sequence
  Synthetic polynucleotide
attaatcctggaagtggtggtact

SEQ ID NO: 285 - DNA, 45 bp, Artificial Sequence
  Synthetic polynucleotide
gcaagatcatacttcggtagaagctacccctatactatggactac

SEQ ID NO: 286 - DNA, 30 bp, Artificial Sequence
  Synthetic polynucleotide
caaagtgttgattatgatggtgataattat

SEQ ID NO: 287 - DNA, 9 bp, Artificial Sequence
  Synthetic polynucleotide
gctgcatcc

SEQ ID NO: 288 - DNA, 27 bp, Artificial Sequence
  Synthetic polynucleotide
cagcaaagtaatgaggatccattcacg

SEQ ID NO: 289 - DNA, 24 bp, Artificial Sequence
  Synthetic polynucleotide
ggctacacattcactgattatgct

SEQ ID NO: 290 - DNA, 24 bp, Artificial Sequence
  Synthetic polynucleotide
attagtacatactctggtaataca

SEQ ID NO: 291 - DNA, 39 bp, Artificial Sequence
  Synthetic polynucleotide
gcaagaaggggcgattacagcctctatgctatggactac

SEQ ID NO: 292 - DNA, 36 bp, Artificial Sequence
  Synthetic polynucleotide
caaagtgttttattcagttcaaatcagaaaaactac

SEQ ID NO: 293 - DNA, 9 bp, Artificial Sequence
  Synthetic polynucleotide
tgggcatcc

SEQ ID NO: 294 - DNA, 24 bp, Artificial Sequence
  Synthetic polynucleotide
catcaatacctctcctcgcgcacg

SEQ ID NO: 295 - DNA, 24 bp, Artificial Sequence
  Synthetic polynucleotide
ggattcactttcagtagctttgga

SEQ ID NO: 296 - DNA, 24 bp, Artificial Sequence
  Synthetic polynucleotide
attagtagtgacagtaggaccatc

SEQ ID NO: 297 - DNA, 33 bp, Artificial Sequence; identical to SEQ ID NO: 273
  Synthetic polynucleotide

SEQ ID NO: 298 - DNA, 30 bp, Artificial Sequence
  Synthetic polynucleotide
gaaagtgttgataattatggcattagtttt

SEQ ID NO: 299 - DNA, 9 bp, Artificial Sequence
  Synthetic polynucleotide
gctgcatcc

SEQ ID NO: 300 - DNA, 27 bp, Artificial Sequence
  Synthetic polynucleotide
cagcaaagtaaggaggttccgctcacg

SEQ ID NO: 301 - DNA, 24 bp, Artificial Sequence
  Synthetic polynucleotide
ggattccctttcagtagctctgcc

SEQ ID NO: 302 - DNA, 21 bp, Artificial Sequence
  Synthetic polynucleotide
attaatagtgatggtaacacc

SEQ ID NO: 303 - DNA, 39 bp, Artificial Sequence
  Synthetic polynucleotide
acaagaaacggggactataggtacgacgagtttgcttac

SEQ ID NO: 304 - DNA, 21 bp, Artificial Sequence
  Synthetic polynucleotide
tcaagtgtaagttccagttac

SEQ ID NO: 305 - DNA, 9 bp, Artificial Sequence
  Synthetic polynucleotide
agcacatcc

SEQ ID NO: 306 - DNA, 27 bp, Artificial Sequence
  Synthetic polynucleotide
caccagtatcatcgttccccacccacg

SEQ ID NO: 307 - DNA, 24 bp, Artificial Sequence
  Synthetic polynucleotide
ggctacacctttactggctactgg

SEQ ID NO: 308 - DNA, 24 bp, Artificial Sequence
  Synthetic polynucleotide
attaatcctagcactggttatact

SEQ ID NO: 309 - DNA, 36 bp, Artificial Sequence
  Synthetic polynucleotide
gcaagagaggggattactactgtgctggttgactac

SEQ ID NO: 310 - DNA, 36 bp, Artificial Sequence; identical to SEQ ID NO: 292
  Synthetic polynucleotide

SEQ ID NO: 311 - DNA, 9 bp, Artificial Sequence
  Synthetic polynucleotide
tgggcatcc

SEQ ID NO: 312 - DNA, 24 bp, Artificial Sequence
  Synthetic polynucleotide
catcaatacctctcctcgcgcacg

SEQ ID NO: 313 - DNA, 24 bp, Artificial Sequence
  Synthetic polynucleotide
ggttactctttcactggctacaat

SEQ ID NO: 314 - DNA, 24 bp, Artificial Sequence
  Synthetic polynucleotide
attgatccttactatggtggttct

SEQ ID NO: 315 - DNA, 42 bp, Artificial Sequence
  Synthetic polynucleotide
gcaagagagaggtcgggctacgttttctctgctatggactac

SEQ ID NO: 316 - DNA, 36 bp, Artificial Sequence; identical to SEQ ID NO: 292
  Synthetic polynucleotide

SEQ ID NO: 317 - DNA, 9 bp, Artificial Sequence
  Synthetic polynucleotide
tgggcatcc

SEQ ID NO: 318 - DNA, 24 bp, Artificial Sequence
  Synthetic polynucleotide
catcaatacctctcctcgcgcacg

SEQ ID NO: 319 - DNA, 24 bp, Artificial Sequence
  Synthetic polynucleotide
ggttactcattcactggctacacc

SEQ ID NO: 320 - DNA, 24 bp, Artificial Sequence
  Synthetic polynucleotide
attaatccttacaatggtgttact

SEQ ID NO: 321 - DNA, 48 bp, Artificial Sequence
  Synthetic polynucleotide
acaagagatcccctttactacggctacagggactctactatggactac

SEQ ID NO: 322 - DNA, 33 bp, Artificial Sequence; identical to SEQ ID NO: 226
  Synthetic polynucleotide

SEQ ID NO: 323 - DNA, 9 bp, Artificial Sequence
  Synthetic polynucleotide
aaagtttcc

SEQ ID NO: 324 - DNA, 27 bp, Artificial Sequence
  Synthetic polynucleotide
tctcaaagtacacatgttccttacacg

SEQ ID NO: 325 - DNA, 24 bp, Artificial Sequence
  Synthetic polynucleotide
ggctacacctttactagctacacg

SEQ ID NO: 326 - DNA, 24 bp, Artificial Sequence
  Synthetic polynucleotide
attaatcctagcagtacgtatact

SEQ ID NO: 327 - DNA, 30 bp, Artificial Sequence; identical to SEQ ID NO: 231
  Synthetic polynucleotide

SEQ ID NO: 328 - DNA, 18 bp, Artificial Sequence
  Synthetic polynucleotide
cagggcattagaggtaat

SEQ ID NO: 329 - DNA, 9 bp, Artificial Sequence
  Synthetic polynucleotide
tccacatcc

SEQ ID NO: 330 - DNA, 27 bp, Artificial Sequence
  Synthetic polynucleotide
ctacagcgtaatgcgtatcctctcacg

SEQ ID NO: 331 - DNA, 24 bp, Artificial Sequence
  Synthetic polynucleotide
ggattcactttcagtagttttgcc

SEQ ID NO: 332 - DNA, 21 bp, Artificial Sequence
  Synthetic polynucleotide
attagaagtggtggtattacc

SEQ ID NO: 333 - DNA, 39 bp, Artificial Sequence
  Synthetic polynucleotide
gcaagagttagtacggctacgtactatggtatggactac

SEQ ID NO: 334 - DNA, 325 bp, Artificial Sequence
  Synthetic polynucleotide
caaattgttctcacccagtctccagcaatcatgtctgcatctctaggggaacgggtcaccatgacctgcactgccagctccagtgtaagttccacttactttcactggtaccaacagaagccaggatcctcccccaaactctggatttatagcacatccaacctggcttctggagtcccacgtcgcttcagtggcagtgcgtctgggacctcttactctctcacaatcagcagcatggaggctgaagatgctgccacttattattgccaccagtatcatcgttccccgctcacgttcggtgctgggaccaagctggagctgaaac

SEQ ID NO: 335 - DNA, 349 bp, Artificial Sequence
  Synthetic polynucleotide
caggtccagctgcagcagtctgcagctgaactggcaagacctggggcctcagtgaagatgtcctgcaaggcttctggctacacctttactacctacacgatgcactgggtaaaacagaggcctggacagggtctggaatggattggattcattaatcctagcagtggatatactgactacaatcagaagttcaaggacaggaccacattgactgcagacaaatcctccagcacagtctacatgcaactgagtagcctgacatctgaggactctgcggtctattactgtgcaaacggggattactacgtcgcttactggggccaagggactctggtcactgtctctgcag

SEQ ID NO: 336 - DNA, 322 bp, Artificial Sequence
  Synthetic polynucleotide
gacatccagatgactcagtctccagcctccctatctgcatctgtgggagaaactgtcaccatcacatgtcgaataagcgagaatatttacagttatttagcatggtatcagcagaaacagggaaaatctcctcagctcctggtctataatgcaaaaatcttagtagaaggtgtgccatcaaggttcagtggcagtggatcaggcacacagttttctctgaagatcaacagcctgcagcctgaagattttgggaattattactgtcaacatcattatactgttccgtggacgttcggtggaggcaccaaactggaaatcaaac

SEQ ID NO: 337 - DNA, 352 bp, Artificial Sequence
  Synthetic polynucleotide
gaagtgaagcttgaggagtctggaggaggcttggtgcaacctggaggatccatgaaactctcctgtgttgcctctggtttcactttcagtgattactggatgaactgggtccgccagtctccagagaaggggcttgaatgggttgctcaaattagattgaaatctgataattatgcaacacattatgcggagtctgtgaaagggaggttcaccatctcaagagatgattccaaaagaagtgtctacctgcaaatgaacaacttaagggctgaagacactggaacttattactgcaatgatggccccccctcggggtgttggggccaaggcaccactctcatagtctcctcag

SEQ ID NO: 338 - DNA, 322 bp, Artificial Sequence
  Synthetic polynucleotide
gacatccagatgactcagtctccagcctccctatctgcatctgtgggagaaactgtcaccatcacatgtcgaataagtgagaatatttacagttatttagcatggtatcagcagaaacagggaaaatctcctcagctcctggtctataatgcaaaaatcttagtagaaggtgtgccatcaaggttcagtggcagtggatcaggcacacagttttctctgaagatcaacagcctgcagcctgaagattttgggaattattactgtcaacatcattatactgttccgtggacgttcggtggaggcaccaaactggaaatcaaac

SEQ ID NO: 339 - DNA, 352 bp, Artificial Sequence
  Synthetic polynucleotide
gaagtgaagcttgaggagtctggaggaggcttggtgcaacctggaggatccatgaaactctcctgtgttgcctctggattcactttcagtaattactggatgaactgggtccgccagtctccagagaaggggcttgaatgggttgctcaaattagattgaaatctgataattatgcaacacattatgcggagtctgtgaaagggaggttcaccatctcaagagatgattccaaaagaagtgtctacctgcaaatgaacaacttaagggctgaagacactggaacttattactgcaatgatggccccccctcggggtgttggggccaaggcaccactctcatagtctcctcag

SEQ ID NO: 340 - DNA, 337 bp, Artificial Sequence
  Synthetic polynucleotide
gatgttgtgatgacccaaactccactctccctgcctgtcagtcttggagatcaagcctccatctcttgcagatctagtcagagccttgtacacagtgatggaaacacctatttaaattggtacctgcagaagccaggccagtctccaaagctcctgatctacaaagtttccaaccgtttttctggggtcccagacaggttcagtggcagtggatcagggacagatttcacactcaagatcaggagagtggaggctgaggatctgggagtttatttctgctctcaaagtacacatgttccttacacgttcggaggggggaccaagctggaaataaaac

SEQ ID NO: 341 - DNA, 352 bp, Artificial Sequence
  Synthetic polynucleotide
caggtccagttgcagcagtctggggctgaactggcaagacctggggcctcagtgaagatgtcctgcaaggcttctggctacacctttactagctacacgatgcactggataaaacagagacctggacagggtcaggaatggattggatacattaatcctagcagtacttatactcattacattaagaaattcaaggacaaggccacattgactgcagacaaatcctccagcacagcctacatgcaactgcgcagcctgacatctgaggactctgcagtctattactgttcaagaggggaactgggagggtttgcttactggggccaagggactctggtcactgtctctgcag

SEQ ID NO: 342 - DNA, 337 bp, Artificial Sequence
  Synthetic polynucleotide
gatgttttgatgacccaaactccactctccctgcctgtcagtcttggagatcaaccctccatctcttgcagatctagtcagagcattgtacatagtaatggaaacacctatttagattggtacctgcagaaaccaggccagtctccaaagctcctgatctacaaagtttccaaccgattttctggggtcccagacaggttcagtggcagtggatcagggacagatttcacactcaagatcagcagagtggaggctgaggatctgggagtttattactgctttcaaggttcacatgttccattcacgttcggctcggggacaaggttggaaataaaac

SEQ ID NO: 343 - DNA, 361 bp, Artificial Sequence
  Synthetic polynucleotide
gaagtccagctgcagcagtctggacctgagctggtaaagcctggggcttcagtgaagatgtcctgcaaggcttctggatacatattcactcactatattatgcactgggtgaagcagaagcctgggcagggccttgagtggattggatgtattaatccttacaatgatggtactaagtacaatgagaagttcaaaggcaaggccacactgacttcagacaaatcctccagcacagcctacatggagctcagcagcctgacctctgaggactctgcggtctattactgtgcaagatactacggctacccttactattctatggactactggggtcaaggaacctcagtcaccgtctcctcag

SEQ ID NO: 344 - DNA, 337 bp, Artificial Sequence
  Synthetic polynucleotide
gccattgtgatgttccagtctccatcctccctggttgtgtcagcaggagagaaggtcactatgagctgcaaatccagtcagagtctgctcaacagtagaacccgaaagaactacttggcttggtaccagcagaaaccagggcagtctcctaaactgctgatctactgggcatccactagggaatctggggtccctgatcgcttcacaggcagtggatctgggacagatttcactctcaccatcagcagtgtgcaggctgaagacctggcagtttattactgcaagcaatcttattatctgtacacgttcggaggggggaccaagctggaaataaaac

SEQ ID NO: 345 - DNA, 352 bp, Artificial Sequence
  Synthetic polynucleotide
gatgtgcagcttcaggagtcaggacctggcctcgtgaaatcttctcagtctctgtctctcacctgctctgtcactggctactccatcaccagtggttattactggaaatggatccggcagtttccaggaaacaaactggaatggatgggctacatcagctacgatggtggcattaactacaacccatctctcaaaaatcgaatctccatcactcgtgacacatctaagaaccagtttttcctgaagttgaattctgtgactactgaggacacagccaaatattactgtgcaagatttggtaagggggctatggactactggggtcaaggaacctcagtcaccgtctcctcag

SEQ ID NO: 346 - DNA, 325 bp, Artificial Sequence
  Synthetic polynucleotide
caaattgttctcacccagtctccagcaatcatgtctgcatctctgggggaccgggtcaccatgacctgcactgccagctcaagtgtaagttccagttacttgcactggtaccagcagaagccaggatcctcccccaaactctggatttatagcacatccaacctggcttctggagtcccagctcgcttcagtggcagtgggtctgggacctcttactctctcacaatcagcagcatggaggctgaagatgctgccacttattactgccaccagtatcatcgttccccacccacgttcggctcggggacaaagttggaaataaaac

SEQ ID NO: 347 - DNA, 358 bp, Artificial Sequence
  Synthetic polynucleotide
gaggtccagctgcaacagtctggacctgagctggtgaagcctggagcttcaatgaagatatcctgcaaggcttctggttactcattcactggctacaccatgaactgggtgaagcagagccatggaaagaaccttgagtggattggacttattaatccttacaatggtggtactaactacaaccagaagttcaagggcaaggccacattaactgtagacaagtcatccagcacagcctacatggagctcctcagtctgacatctgaggactctgcagtctattactgtgcaagaggggtctatgattacgacggatttacttactggggccaagggactctggtcactgtctctgcag

SEQ ID NO: 348 - DNA, 337 bp, Artificial Sequence
  Synthetic polynucleotide
gatgttgtgatgacccaaactccactctccctgcctgtcagtcttggagatcaagcctccatctcttgcagatctagtcagagccttgtacacagtgatggaaacacctatttatattggtacctgcagaagccaggccagtctccaaagctcctgatctacaaagtttccaaccgattttctggggtcccagacaggttcagtggcagtggatcagggacagatttcacactcaagatcagcagagtggaggctgaggatctgggagtttatttctgctctcaaagtacacatgttccttacacgttcggaggggggaccaagctggaaataaaac

SEQ ID NO: 349 - DNA, 352 bp, Artificial Sequence
  Synthetic polynucleotide
caggtccagctgcagcagtctggggctgaactggcaagacctggggcctcagtgaagatgtcctgcaaggcttctggctacacctttactacctacacgatgcactggttaaaacagaggcctggacagggtctggaatggattggatacattaatcctcgcagtggttatagtaattacaatcagaagttcaaggacaaggccacattgactgcagacaagtcctccaacacagcctacatgcaactgaacaccctgacatctgaggactctaaagtctattactgttcaagaggggaactgggagggtttgcttactggggccaagggactctggtcactgtctctgcag

SEQ ID NO: 350 - DNA, 322 bp, Artificial Sequence
  Synthetic polynucleotide
gacattcagatgacccagtctcctgcctcccagtctgcatctctgggagaaagtgtcaccatcacatgcctggcaagtcagaccattggtacatggttagcatggtatcagcagaaaccagggaaatctcctcagctcctgatttatgctgcagccagcttggcagatggggtcccatcaaggttcagtggtagtggatctggcacaagattttctttcaagatcagcagcctacaggctgaagattttgtaagttattactgtcaacaactttacagtattcctcggacgttcggtggaggcaccaagctggaaatcaaac

SEQ ID NO: 351 - DNA, 352 bp, Artificial Sequence
  Synthetic polynucleotide
gaggtccagctgcaacagtctggacctgagctggtgaagcctggggcttcagtgaagatgtcctgcaaggcttctggatacagattcactgactacaacatgcactgggtgaagcagagccatggaaagagccttgagtggattggatatattaaccctaacaatggtggtactaactacaaccaaaacttcaagggcaaggccacattgactgtgaacaagtcctccagcacagcctacatggagctccgcagcctgacatcggaggattctgcagcctattactgtgcaagagattacttgtacttctttgactgctggggccaaggcaccactctcacagtctcctcag

SEQ ID NO: 352 - DNA, 337 bp, Artificial Sequence
  Synthetic polynucleotide
gatgttgtgatgacccaaactccactctccctgcctgtcagtcttggagatcaagcctccatctcttgcagagctagtcagagccttgtacacagtaatggaaacacctatttacattggttcctgcagaagccaggccagtctccaaagctcctgatctacaaagtttccaaccgattttctggggtcccagacaggttcagtggcagtggatcacggacagatttcacactcaagatcagcagagtggaggctgaggatctgggagtttatttctgctctcaaattacacatgttccgtacacgttcggaggggggaccaagctggaaataaaac

SEQ ID NO: 353 - DNA, 352 bp, Artificial Sequence
  Synthetic polynucleotide
caaatccagttggtgcagtctggacctgcgctgaagaagcctggagagacagtcaagatctcctgcaaggcttctggttataccttcacagactattcaatgcactggataaagcaggctccaggaaagggtttaaagtggatgggctggataagcactgagactggtgagccaacatatgcagatggcttcaagggacggtttgacttctctttggaaacctctgccgacactgcctatttgtccatcaacaacctcacaaatgaggacacggctacatatttctgtactagaggtctatggtcctcgtttgcttactggggccaagggactctggtcactgtctctgcag

SEQ ID NO: 354 - DNA, 334 bp, Artificial Sequence
  Synthetic polynucleotide
gacattgtgctgacacagtctcctgcttccttagctgtatctctggggcagagggccaccatctcatgcagggccagcaaaagtgtcagtacatctggctatagttatatacactggtaccaacagaaaccaggacagccacccaaactcctcatctatcttgcatccaacctagaatctggggtccctgccaggttcagtggcagtgggtctgggacagacttcaccctcaacatccatcctgtggaggaggaggatgctgcaacctattactgtcagcacagtagggagcttccgctcacgttcggtgctgggaccaagctggagctgaaac

SEQ ID NO: 355 - DNA, 355 bp, Artificial Sequence
  Synthetic polynucleotide
gatgtgcagctggtggagtctgggggaggcttggtgcagcctagagggtcccggaaactctcctgtgcagcctctggattcactttcagtagctttggaatgcactgggttcgtcaggctccagagaaggggctggagtgggtcgcatacattagtagtgacagtaggaccatctattatgcagacacagtgaagggccgattcaccatctccagagacaatcccacgaacaccctgttcctgcaaatgaccagtctcaggtctgaggacacggccatgtattactgtgcaagagactacggtagaacctacgaggcttactggggccaagggactctggtcactgtctctgcag

SEQ ID NO: 356 - DNA, 322 bp, Artificial Sequence
  Synthetic polynucleotide
gacatccagatgattcagtctccatcgtccatgtttgcctctctgggagacagagtcagtctctcttgtcgggctagtcaggacattggaggaaatttagactggtatcagcagaaaccaggtggaactattaaactcctgatctactccacatccaatttaaattctggtgtcccatcaaggttcagtggcagtgggtctgggtcagattattctctcaccatcaccagcctggagtctgaagattttgcagactattactgtctacagcgtaatgcgtatccgctcactttcggtgctgggaccaagctggagctgaaac

SEQ ID NO: 357 - DNA, 355 bp, Artificial Sequence
  Synthetic polynucleotide
gaagtgaaactgatggagtctgggggagacttagtgaagcctggagggtccctgaaactctcctgtgcagcctctggattcactttcagtagttatgccatgtcttgggttcgccagactccagagaagaggctggagtgggtcgcgtccattagaagtggtggtaccacctactatccagacagtgtgaagggccgattcaccatctccagagataatgccaggaacatcctgtacctgcgaatgagtagtctgaggtctgaggacacggccatatattactgtgcaaaagtgggcggtaacccctatcctatggactactggggtcaaggaacctcagtcaccgtctcctcag

SEQ ID NO: 358 - DNA, 325 bp, Artificial Sequence
  Synthetic polynucleotide
gaaattgtgctcacccagtctccaaccaccatggctgcatctcccggggagaagatcactatcacctgcagtgccagctcaagtataagttccaattacttgcattggtatcagcagaagccaggattctcccctaaactcttgatttataggacatccaatctggcttctggagtcccagctcgcttcagtggcagtgggtctgggacctcttactctctcacaattggcaccatggaggctgaagatgttgccacttactactgccagcagggtagtagtataccgctcacgttcggtgctgggaccaagctggagctgaaac

SEQ ID NO: 359 - DNA, 367 bp, Artificial Sequence
  Synthetic polynucleotide
caggtccagctgcagcagtctggagctgagctggtaaggcctgggacttcagtgaaggtgtcctgcaaggcttctggatacgccttcagtaattacttgatagagtgggttaagcagaggcctggacagggccttgagtggattggagtgattaatcctggaagtggtggtactaactacaatgagaagttcaagggcaaggcaacaatgactgcagacaaatcctccagcactgcctacatgcacctcagcaacctgacatctgaggactctgtggtctatttctgtgcaagatcatacttcggtagaagctacccctatactatggactactggggtcaaggaacctcagtcaccgtctcctcag

SEQ ID NO: 360 - DNA, 334 bp, Artificial Sequence
  Synthetic polynucleotide
gatattgtgctgacccaatctccagcttctttggctgtgtctctagggcagagggccaccatctcctgcaaggccagccaaagtgttgattatgatggtgataattatgtgaactggtaccaacagaaagtaggacagccacccaaactcctcatctctgctgcatccaatctagaatctgggatcccagccaggtttagtggcagtgggtctgggacagacttcaccctcaacatccatcctgtggaggaggaggatgctgcaacctattactgtcagcaaagtaatgaggatccattcacgttcggctcggggacaaagttggaaataaaac

SEQ ID NO: 361 - DNA, 361 bp, Artificial Sequence
  Synthetic polynucleotide
caggtccagctgcagcagtctgggcctgagctggtgaggcctggggtctcagtgaagatttcctgcaagggttccggctacacattcactgattatgctatgcactgggtgaagcagagtcatgcaaagagtctagagtggattggagttattagtacatactctggtaatacaaactacaaccagaagtttcaggacaaggccaccatgactgtagacaaatcctccagcacagcctatatggcacttgccagattgacatctgacgattctgccatctattactgtgcaagaaggggcgattacagcctctatgctatggactactggggtcaaggaacctcagtcaccgtctcctcag

SEQ ID NO: 362 - DNA, 337 bp, Artificial Sequence
  Synthetic polynucleotide
aacattatgatgacacagtcgccatcatctctggctgtgtctgcaggagaaaaggtcactatgagctgtaagtccagtcaaagtgttttattcagttcaaatcagaaaaactacttggcctggtaccagcagaaaccagggcagtctcctagactgctgatctactgggcatccactagggaatctggtgtccctgatcgcttcacaggcagtggatctgggacagattttactcttaccatcagcaatgttcaagctgaagacctggcagtttattactgtcatcaatacctctcctcgcgcacgttcggtgctgggaccaagctggagctgaaac

SEQ ID NO: 363 - DNA, 355 bp, Artificial Sequence; identical to SEQ ID NO: 355
  Synthetic polynucleotide

SEQ ID NO: 364 - DNA, 334 bp, Artificial Sequence
  Synthetic polynucleotide
gacattgtgctgacccaatctccagcttctttggctctgtctctagggcagagggccaccatctcctgcagagccagcgaaagtgttgataattatggcattagttttatgaactggttccaacagaaacccggacagccacccaaactcctcatctatgctgcatccaaccaaggatccggggtccctgccaggtttagtggcagtgggtctgggacagacttcagcctcaacatccatcctatggaggaggatgatactgcaatgtatttctgtcagcaaagtaaggaggttccgctcacgttcggtgctgggaccaagctggagctgaaac

SEQ ID NO: 365 - DNA, 358 bp, Artificial Sequence
  Synthetic polynucleotide
gaagtgaggctggtggagtctgggggaggcttgatgcagcctggagggtccctgaaactcccctgtgcagcctctggattccctttcagtagctctgccatgtcttgggttcgccagactccagagaagaggctggagtgggtcgcatccattaatagtgatggtaacacctactatcccgacagtgtgaagggccgattcaccatctccagagatagtgccaggaacatcctgtacctccaaatgagcagtctgaggtctgaggacacggccatgtattactgtacaagaaacggggactataggtacgacgagtttgcttactggggccaagggactctggtcactgtctctgcag

SEQ ID NO: 366 - DNA, 325 bp, Artificial Sequence
  Synthetic polynucleotide
caaattgttctcacccagtctccagcaatcatgtctgcatctctaggggaacgggtcaccatgacctgcactgccagctcaagtgtaagttccagttacttgcactggtaccagcagaagccaggatcctcccccaaactctggatttatagcacatccaacctggcttctggagtcccagctcgcttcagtggcagtgggtctgggacctcttactctctcacaatcagcagcatggaggctgaagatgctgccacttattactgccaccagtatcatcgttccccacccacgttcggagctgggaccaagctggagctgaaac

SEQ ID NO: 367 - DNA, 358 bp, Artificial Sequence
  Synthetic polynucleotide
caggtccagcttcagcagtctggggctgaactggcaaaacctggggcctcagtgaagatgtcctgcaaggcttctggctacacctttactggctactggatgcactgggtaaaacagaggcctggacagggtctggaatggcttggatacattaatcctagcactggttatactgagtccaatcagaagttcaaggacaaggccacattgactgcagacaaatcctccaccacagcctacatgcaactgagaagcctgacacctgaggactctgcagtctattactgtgcaagagaggggattactactgtgctggttgactactggggccaaggcaccactctcacagtctcctcag

SEQ ID NO: 368 - DNA, 337 bp, Artificial Sequence; identical to SEQ ID NO: 362
  Synthetic polynucleotide

SEQ ID NO: 369 - DNA, 364 bp, Artificial Sequence
  Synthetic polynucleotide
caggtgcagctgaagcagtctggacctgagctggagaagcctggcgcttcagtgaagatatcctgcaaggcttctggttactctttcactggctacaatatgaactgggtgaagcagagcaatggaaagagccttgagtggattggaaatattgatccttactatggtggttctacctacaaccagaagttcacgggcaaggccacattgactgtagacaaatcctccagcacagcctacatgcagctcaagagcctgacatctgaggactctgcagtgtattactgtgcaagagagaggtcgggctacgttttctctgctatggactactggggtcaaggaacctcagtcaccgtctcctcag

SEQ ID NO: 370 - DNA, 337 bp, Artificial Sequence; identical to SEQ ID NO: 362
  Synthetic polynucleotide

SEQ ID NO: 371 - DNA, 370 bp, Artificial Sequence
  Synthetic polynucleotide
gaggtccagctgcaacagtctggacctgagctggtgaagcctggaggttcaatgaagatatcctgcaaggcttctggttactcattcactggctacaccatgaactgggtgaagcggagccatggaaagaaccttgagtggattggacttattaatccttacaatggtgttactacctacaaccagaacttcaagggcaaggccacattagctgtagacaagtcatccagcacagcctacatggagctcctcggtctgacatctgaggactctgcagtctattactgtacaagagatcccctttactacggctacagggactctactatggactactggggtcaaggaacctcagtcaccgtctcctcag

SEQ ID NO: 372 - DNA, 337 bp, Artificial Sequence; identical to SEQ ID NO: 340
  Synthetic polynucleotide

SEQ ID NO: 373 - DNA, 352 bp, Artificial Sequence
  Synthetic polynucleotide
gaggtccagctgcagcagtctggggctgaactggcaagacctggggcctcagtgaagatgtcctgcaaggcttctggctacacctttactagctacacgatgcactggataaaacagagacctggacagggtcaggaatggattggatacattaatcctagcagtacgtatactcattacattaagaagttcaaggacaaggccacattgactgcagacaaatcctccagcacagcctacatgcaactgcgcagcctgacatctgaggactctgcagtctattactgttcaagaggggaactgggagggtttgcttactggggccaagggactctggtcactgtctctgcag

SEQ ID NO: 374 - DNA, 322 bp, Artificial Sequence
  Synthetic polynucleotide
gacatccagatgattcagtctccatcgtccatgtttgcctctctgggagacagagtcagtctctcttgtcgggctagtcagggcattagaggtaatttagactggtatcagcagaaaccaggtggaactattaaactcctgatctactccacatccattttaaattctggtgtcccatcaaggttcagtggcagtgggtctgggtcagattattctctcaccatcaccagcctagagtctgaagattttgcagactattactgtctacagcgtaatgcgtatcctctcacgttcggttctgggaccaagctggagctgaaac

SEQ ID NO: 375 - DNA, 358 bp, Artificial Sequence
  Synthetic polynucleotide
gaagtgaagttggtggagtctgggggaggcttaatgaagcctggagggtccctgaaactctcctgtgcggcctctggattcactttcagtagttttgccttgtcttgggttcgccagactccagagaagaggctggagtgggtcgcatccattagaagtggtggtattacctaccatgcagacagtgtgaagggccgattcaccatctccagagataatgccgggaacatcctgtacctgcaaatgaacagtctgaggtctgaggacacggccatgtatttctgtgcaagagttagtacggctacgtactatggtatggactactggggtcaaggaacctcagtcaccgtctcctcag

SEQ ID NO: 376 - protein, 116 aa, Artificial Sequence
  Synthetic peptide
QVQLVQSGAEVKKPGASVKVSCKASGYTFTTYTMHWVRQAPGQGLEWMGFINPSSGYTDYAQKFQGRVTMTRDTSTSTVYMELSSLRSEDTAVYYCARGDYYVAYWGQGTLVTVSS

SEQ ID NO: 377 - protein, 116 aa, Artificial Sequence
  Synthetic peptide
QVQLVQSGAEVKKPGASVKVSCKASGYTFTTYTMHWVRQAPGQGLEWMGFINPSSGYTDYAQKFQGRVTMTADTSTSTVYMELSSLRSEDTAVYYCANGDYYVAYWGQGTLVTVSS

SEQ ID NO: 378 - protein, 116 aa, Artificial Sequence
  Synthetic peptide
QVQLVQSGAEVKKPGASVKMSCKASGYTFTTYTMHWVRQAPGQGLEWIGFINPSSGYTDYAQKFQGRVTLTADTSTSTVYMELSSLRSEDTAVYYCANGDYYVAYWGQGTLVTVSS

SEQ ID NO: 379 - protein, 116 aa, Artificial Sequence
  Synthetic peptide
QVQLVQSGAEVKKPGASVKMSCKASGYTFTTYTMHWVRQAPGQGLEWIGFINPSSGYTDYAQKFQGRVTLTADKSTSTVYMELSSLRSEDTAVYYCANGDYYVAYWGQGTLVTVSS

SEQ ID NO: 380 - protein, 108 aa, Artificial Sequence
  Synthetic peptide
DIQMTQSPSSLSASVGDRVTITCTASSSVSSTYFHWYQQKPGKAPKLLIYSTSNLASGVPSRFSGSGSGTDFTLTISSLQPEDFATYYCHQYHRSPLTFGQGTKLEIK

SEQ ID NO: 381 - protein, 108 aa, Artificial Sequence
  Synthetic peptide
DIQMTQSPSSLSASVGDRVTITCTASSSVSSTYFHWYQQKPGKAPKLLIYSTSNLASGVPSRFSGSGSGTDYTLTISSLQPEDFATYYCHQYHRSPLTFGQGTKLEIK

SEQ ID NO: 382 - protein, 108 aa, Artificial Sequence
  Synthetic peptide
DIQLTQSPSSLSASVGDRVTMTCTASSSVSSTYFHWYQQKPGKAPKLLIYSTSNLASGVPSRFSGSGSGTDYTLTISSMQPEDAATYYCHQYHRSPLTFGQGTKLEIK

SEQ ID NO: 383 - protein, 108 aa, Artificial Sequence
  Synthetic peptide
DIQLTQSPSSLSASVGDRVTMTCTASSSVSSTYFHWYQQKPGKAPKLWIYSTSNLASGVPSRFSGSGSGTDYTLTISSMQPEDAATYYCHQYHRSPLTFGQGTKLEIK

SEQ ID NO: 384 - protein, 117 aa, Artificial Sequence
  Synthetic peptide
EVQLLESGGGLVQPGGSLRLSCAASGFTFSNYWMNWVRQAPGKGLEWVSQIRLKSDNYATHYADSVKGRFTISRDNSKNTLYLQMNSLRAEDTAVYYCAKGPPSGCWGQGTLVTVSS

SEQ ID NO: 385 - protein, 117 aa, Artificial Sequence
  Synthetic peptide
EVQLLESGGGLVQPGGSMRLSCAASGFTFSNYWMNWVRQAPGKGLEWVAQIRLKSDNYATHYADSVKGRFTISRDDSKNTVYLQMNSLRAEDTGVYYCNDGPPSGCWGQGTLLTVSS

SEQ ID NO: 386 - protein, 117 aa, Artificial Sequence
  Synthetic peptide
EVQLLESGGGLVQPGGSMRLSCAASGFTFSNYWMNWVRQAPGKGLEWVAQIRLKSDNYATHYADSVKGRFTISRDDSKNTVYLQMNSLRAEDTGVYYCNDGPPSGYWGQGTLLTVSS

SEQ ID NO: 387 - protein, 117 aa, Artificial Sequence
  Synthetic peptide
EVQLLESGGGLVQPGGSMRLSCAASGFTFSNYWMNWVRQAPGKGLEWVAQIRLKSDNYATHYADSVKGRFTISRDDSKNTVYLQMNSLRAEDTGVYYCNDGPPSGSWGQGTLLTVSS

SEQ ID NO: 388 - protein, 107 aa, Artificial Sequence
  Synthetic peptide
DIQMTQSPSSLSASVGDRVTITCRISENIYSYLAWYQQKPGKAPKLLIYNAKILVEGVPSRFSGSGSGTDFTLTISSLQPEDFATYYCQHHYTVPWTFGQGTKLEIK

SEQ ID NO: 389 - protein, 107 aa, Artificial Sequence
  Synthetic peptide
DIQMTQSPSSLSASVGDRVTITCRISENIYSYLAWYQQKPGKAPKLLVYNAKILVEGVPSRFSGSGSGTDFTLTISSLQPEDFGTYYCQHHYTVPWTFGQGTKLEIK

SEQ ID NO: 390 - protein, 107 aa, Artificial Sequence
  Synthetic peptide
DIQMTQSPSSLSASVGDRVTITCRISENIYSYLAWYQQKPGKAPKLLVYNAKSLVEGVPSRFSGSGSGTDFTLTISSLQPEDFGTYYCQHHYTVPWTFGQGTKLEIK

SEQ ID NO: 391 - protein, 117 aa, Artificial Sequence
  Synthetic peptide
QVQLVQSGAEVKKPGASVKVSCKASGYTFTSYTMHWVRQAPGQGLEWMGYINPSSTYTHYAQKFQGRVTMTRDTSTSTVYMELSSLRSEDTAVYYCARGELGGFAYWGQGTLVTVSS

SEQ ID NO: 392 - protein, 117 aa, Artificial Sequence
  Synthetic peptide
QVQLVQSGAEVKKPGASVKVSCKASGYTFTSYTMHWVRQAPGQGLEWMGYINPSSTYTHYAQKFQGRVTMTADTSTSTVYMELSSLRSEDTAVYYCSRGELGGFAYWGQGTLVTVSS

SEQ ID NO: 393 - protein, 117 aa, Artificial Sequence
  Synthetic peptide
QVQLVQSGAEVKKPGASVKMSCKASGYTFTSYTMHWIRQAPGQGLEWIGYINPSSTYTHYAQKFQGRATLTADTSTSTAYMELSSLRSEDTAVYYCSRGELGGFAYWGQGTLVTVSS

SEQ ID NO: 394 - protein, 117 aa, Artificial Sequence
  Synthetic peptide
QVQLVQSGAEVKKPGASVKMSCKASGYTFTSYTMHWIRQAPGQGQEWIGYINPSSTYTHYAQKFQGRATLTADTSTSTAYMELSSLRSEDTAVYYCSRGELGGFAYWGQGTLVTVSS

SEQ ID NO: 395 - protein, 117 aa, Artificial Sequence
  Synthetic peptide
QVQLVQSGAEVKKPGASVKMSCKASGYTFTSYTMHWIRQAPGQGLEWIGYINPSSTYTHYAQKFQGRATLTADKSTSTAYMELSSLRSEDTAVYYCSRGELGGFAYWGQGTLVTVSS

SEQ ID NO: 396 - protein, 117 aa, Artificial Sequence
  Synthetic peptide
QVQLVQSGAEVKKPGASVKMSCKASGYTFTSYTMHWIRQAPGQGQEWIGYINPSSTYTHYAQKFQGRATLTADKSTSTAYMELSSLRSEDTAVYYCSRGELGGFAYWGQGTLVTVSS

SEQ ID NO: 397 - protein, 112 aa, Artificial Sequence
  Synthetic peptide
DVVMTQSPLSLPVTLGQPASISCRSSQSLVHSDGNTYLNWFQQRPGQSPRRLIYKVSNRFSGVPDRFSGSGSGTDFTLKISRVEAEDVGVYYCSQSTHVPYTFGQGTKLEIK

SEQ ID NO: 398 - protein, 112 aa, Artificial Sequence
  Synthetic peptide
DVVMTQSPLSLPVTLGQPASISCRSSQSLVHSDGNTYLNWYQQRPGQSPRLLIYKVSNRFSGVPDRFSGSGSGTDFTLKISRVEAEDVGVYYCSQSTHVPYTFGQGTKLEIK

SEQ ID NO: 399 - protein, 112 aa, Artificial Sequence
  Synthetic peptide
DVVMTQSPLSLPVTLGQPASISCRSSQSLVHSEGNTYLNWYQQRPGQSPRLLIYKVSNRFSGVPDRFSGSGSGTDFTLKISRVEAEDVGVYYCSQSTHVPYTFGQGTKLEIK

SEQ ID NO: 400 - protein, 112 aa, Artificial Sequence
  Synthetic peptide
DVVMTQSPLSLPVTLGQPASISCRSSQSLVHSSGNTYLNWYQQRPGQSPRLLIYKVSNRFSGVPDRFSGSGSGTDFTLKISRVEAEDVGVYYCSQSTHVPYTFGQGTKLEIK

SEQ ID NO: 401 - protein, 112 aa, Artificial Sequence
  Synthetic peptide
DVVMTQSPLSLPVTLGQPASISCRSSQSLVHSEGSTYLNWYQQRPGQSPRLLIYKVSNRFSGVPDRFSGSGSGTDFTLKISRVEAEDVGVYYCSQSTHVPYTFGQGTKLEIK

SEQ ID NO: 402 - protein, 112 aa, Artificial Sequence
  Synthetic peptide
DVVMTQSPLSLPVTLGQPASISCRSSQSLVHSSGSTYLNWYQQRPGQSPRLLIYKVSNRFSGVPDRFSGSGSGTDFTLKISRVEAEDVGVYYCSQSTHVPYTFGQGTKLEIK

SEQ ID NO: 403 - protein, 117 aa, Artificial Sequence
  Synthetic peptide
QVQLVQSGAEVKKPGASVKVSCKASGYRFTDYNMHWVRQAPGQGLEWMGYINPNNGGTNYAQKFQGRVTMTRDTSTSTVYMELSSLRSEDTAVYYCARDYLYFFDCWGQGTLVTVSS

SEQ ID NO: 404 - protein, 117 aa, Artificial Sequence
  Synthetic peptide
QVQLVQSGAEVKKPGASVKVSCKASGYRFTDYNMHWVRQAPGQGLEWMGYINPNNGGTNYAQKFQGRVTMTVDTSTSTVYMELSSLRSEDTAVYYCARDYLYFFDCWGQGTLVTVSS

SEQ ID NO: 405 - protein, 117 aa, Artificial Sequence
  Synthetic peptide
QVQLVQSGAEVKKPGASVKMSCKASGYRFTDYNMHWVRQAPGQGLEWIGYINPNNGGTNYAQKFQGRATLTVDTSTSTAYMELSSLRSEDTAVYYCARDYLYFFDCWGQGTLLTVSS

SEQ ID NO: 406 - protein, 117 aa, Artificial Sequence
  Synthetic peptide
QVQLVQSGAEVKKPGASVKMSCKASGYRFTDYNMHWVRQAPGQGLEWIGYINPNNGGTNYAQKFQGRATLTVDKSTSTAYMELSSLRSEDTAVYYCARDYLYFFDCWGQGTLLTVSS

SEQ ID NO: 407 - protein, 117 aa, Artificial Sequence
  Synthetic peptide
QVQLVQSGAEVKKPGASVKMSCKASGYRFTDYNMHWVRQAPGQGLEWIGYINPNNGGTNYAQKFQGRATLTVNKSTSTAYMELSSLRSEDTAVYYCARDYLYFFDCWGQGTLLTVSS

SEQ ID NO: 408 - protein, 117 aa, Artificial Sequence
  Synthetic peptide
QVQLVQSGAEVKKPGASVKMSCKASGYRFTDYNMHWVRQAPGQGLEWIGYINPNNGGTNYAQKFQGRATLTVNTSTSTAYMELSSLRSEDTAVYYCARDYLYFFDCWGQGTLLTVSS

SEQ ID NO: 409 - protein, 107 aa, Artificial Sequence
  Synthetic peptide
DIQMTQSPSSLSASVGDRVTITCLASQTIGTWLAWYQQKPGKAPKLLIYAAASLADGVPSRFSGSGSGTDFTLTISSLQPEDFATYYCQQLYSIPRTFGQGTKLEIK

SEQ ID NO: 410 - protein, 107 aa, Artificial Sequence
  Synthetic peptide
DIQMTQSPSSLSASVGDRVTITCLASQTIGTWLAWYQQKPGKAPKLLIYAAASLADGVPSRFSGSGSGTDFTFTISSLQPEDFVTYYCQQLYSIPRTFGQGTKLEIK

SEQ ID NO: 411 - protein, 107 aa, Artificial Sequence
  Synthetic peptide
DIQMTQSPSSLSASVGDRVTITCRASQTIGTWLAWYQQKPGKAPKLLIYAAASLADGVPSRFSGSGSGTDFTFTISSLQPEDFVTYYCQQLYSIPRTFGQGTKLEIK

SEQ ID NO: 412 - protein, 118 aa, Artificial Sequence
  Synthetic peptide
EVQLVESGGGLVQPGGSLRLSCAASGFTFSSFGMHWVRQAPGKGLEWVSYISSDSRTIYYADSVKGRFTISRDNAKNSLYLQMNSLRAEDTAVYYCARDYGRTYEAYWGQGTLVTVSS

SEQ ID NO: 413 - protein, 118 aa, Artificial Sequence
  Synthetic peptide
EVQLVESGGGLVQPGGSLRLSCAASGFTFSSFGMHWVRQAPGKGLEWVAYISSDSRTIYYADSVKGRFTISRDNAKNSLYLQMNSLRAEDTAVYYCARDYGRTYEAYWGQGTLVTVSS

SEQ ID NO: 414 - protein, 111 aa, Artificial Sequence
  Synthetic peptide
DIVMTQSPDSLAVSLGERATINCRASKSVSTSGYSYIHWYQQKPGQPPKLLIYLASNLESGVPDRFSGSGSGTDFTLTISSLQAEDVAVYYCQHSRELPLTFGQGTKLEIK

SEQ ID NO: 415 - protein, 111 aa, Artificial Sequence
  Synthetic peptide
DIVLTQSPDSLAVSLGERATINCRASKSVSTSGYSYIHWYQQKPGQPPKLLIYLASNLESGVPDRFSGSGSGTDFTLTISSVQAEDVAVYYCQHSRELPLTFGQGTKLELK

SEQ ID NO: 416 - protein, 121 aa, Artificial Sequence
  Synthetic peptide
QVQLVQSGAEVKKPGASVKVSCKASGYSFTGYNMNWVRQAPGQGLEWMGNIDPYYGGSTYAQKFQGRVTMTRDTSTSTVYMELSSLRSEDTAVYYCARERSGYVFSAMDYWGQGTLVTVSS

SEQ ID NO: 417 - protein, 121 aa, Artificial Sequence
  Synthetic peptide
QVQLVQSGAEVKKPGASVKVSCKASGYSFTGYNMNWVRQAPGQGLEWMGNIDPYYGGSTYAQKFQGRVTMTVDTSTSTVYMELSSLRSEDTAVYYCARERSGYVFSAMDYWGQGTLVTVSS

SEQ ID NO: 418 - protein, 121 aa, Artificial Sequence
  Synthetic peptide
QVQLVQSGAEVKKPGASVKISCKASGYSFTGYNMNWVRQAPGQGLEWIGNIDPYYGGSTYAQKFQGRATLTVDTSTSTAYMELSSLRSEDTAVYYCARERSGYVFSAMDYWGQGTLVTVSS

SEQ ID NO: 419 - protein, 121 aa, Artificial Sequence
  Synthetic peptide
QVQLVQSGAEVKKPGASVKISCKASGYSFTGYNMNWVRQAPGQGLEWIGNIDPYYGGSTYAQKFQGRATLTVDKSTSTAYMELSSLRSEDTAVYYCARERSGYVFSAMDYWGQGTLVTVSS

SEQ ID NO: 420 - protein, 112 aa, Artificial Sequence
  Synthetic peptide
DIVMTQSPDSLAVSLGERATINCKSSQSVLFSSNQKNYLAWYQQKPGQPPKLLIYWASTRESGVPDRFSGSGSGTDFTLTISSLQAEDVAVYYCHQYLSSRTFGQGTKLEIK

SEQ ID NO: 421 - protein, 112 aa, Artificial Sequence
  Synthetic peptide
DIVMTQSPDSLAVSLGERVTMNCKSSQSVLFSSNQKNYLAWYQQKPGQPPKLLIYWASTRESGVPDRFSGSGSGTDFTLTISSVQAEDVAVYYCHQYLSSRTFGQGTKLEIK

SEQ ID NO: 422 - protein, 117 aa, Artificial Sequence
  Synthetic peptide
EVQLLESGGGLVQPGGSMRLSCAASGFTFSNYWMNWVRQAPGKGLEWVAQIRLKSDNYATHYADSVKGRFTISRDDSKNTVYLQMNSLRAEDTGVYYCNDGPPSGAWGQGTLLTVSS

SEQ ID NO: 423 - protein, 117 aa, Artificial Sequence
  Synthetic peptide
QVQLVQSGAEVKKPGASVKVSCKASGYTFTSYTMHWVRQAPGQGLEWMGYINPSSTYTHYIKKFKDRVTMTADTSTSTVYMELSSLRSEDTAVYYCSRGELGGFAYWGQGTLVTVSS

SEQ ID NO: 424 - protein, 117 aa, Artificial Sequence
  Synthetic peptide
QVQLVQSGAEVKKPGASVKMSCKASGYTFTSYTMHWIRQAPGQGLEWIGYINPSSTYTHYIKKFKDRATLTADTSTSTAYMELSSLRSEDTAVYYCSRGELGGFAYWGQGTLVTVSS

SEQ ID NO: 425 - protein, 117 aa, Artificial Sequence
  Synthetic peptide
QVQLVQSGAEVKKPGASVKMSCKASGYTFTSYTMHWIRQAPGQGQEWIGYINPSSTYTHYIKKFKDRATLTADTSTSTAYMELSSLRSEDTAVYYCSRGELGGFAYWGQGTLVTVSS

SEQ ID NO: 426 - protein, 117 aa, Artificial Sequence
  Synthetic peptide
QVQLVQSGAEVKKPGASVKMSCKASGYTFTSYTMHWIRQAPGQGLEWIGYINPSSTYTHYIKKFKDRATLTADKSTSTAYMELSSLRSEDTAVYYCSRGELGGFAYWGQGTLVTVSS

SEQ ID NO: 427 - protein, 117 aa, Artificial Sequence
  Synthetic peptide
QVQLVQSGAEVKKPGASVKMSCKASGYTFTSYTMHWIRQAPGQGQEWIGYINPSSTYTHYIKKFKDRATLTADKSTSTAYMELSSLRSEDTAVYYCSRGELGGFAYWGQGTLVTVSS

SEQ ID NO: 428 - protein, 116 aa, Artificial Sequence
  Synthetic peptide
  misc_feature (5)..(5): Xaa can be any naturally occurring amino acid
  misc_feature (8)..(8): Xaa can be any naturally occurring amino acid
  misc_feature (11)..(13): Xaa can be any naturally occurring amino acid
  misc_feature (20)..(20): Xaa can be any naturally occurring amino acid
  misc_feature (31)..(31): Xaa can be any naturally occurring amino acid
  misc_feature (33)..(33): Xaa can be any naturally occurring amino acid
  misc_feature (35)..(35): Xaa can be any naturally occurring amino acid
  misc_feature (38)..(38): Xaa can be any naturally occurring amino acid
  misc_feature (40)..(40): Xaa can be any naturally occurring amino acid
  misc_feature (48)..(48): Xaa can be any naturally occurring amino acid
  misc_feature (50)..(50): Xaa can be any naturally occurring amino acid
  misc_feature (55)..(55): Xaa can be any naturally occurring amino acid
  misc_feature (57)..(57): Xaa can be any naturally occurring amino acid
  misc_feature (59)..(59): Xaa can be any naturally occurring amino acid
  misc_feature (61)..(61): Xaa can be any naturally occurring amino acid
  misc_feature (65)..(68): Xaa can be any naturally occurring amino acid
  misc_feature (70)..(70): Xaa can be any naturally occurring amino acid
  misc_feature (72)..(72): Xaa can be any naturally occurring amino acid
  misc_feature (74)..(76): Xaa can be any naturally occurring amino acid
  misc_feature (79)..(80): Xaa can be any naturally occurring amino acid
  misc_feature (82)..(82): Xaa can be any naturally occurring amino acid
  misc_feature (87)..(87): Xaa can be any naturally occurring amino acid
  misc_feature (90)..(91): Xaa can be any naturally occurring amino acid
  misc_feature (98)..(98): Xaa can be any naturally occurring amino acid
  misc_feature (101)..(101): Xaa can be any naturally occurring amino acid
  misc_feature (116)..(116): Xaa can be any naturally occurring amino acid
QVQLXQSXAEXXXPGASVKXSCKASGYTFTXYXMXWVXQXPGQGLEWXGXINPSXGXTXYXQKFXXXXTXTXDXSXSTXXMXLSSLXSEXXAVYYCAXGDXYVAYWGQGTLVTVSX

SEQ ID NO: 429 - protein, 116 aa, Artificial Sequence
  Synthetic peptide
  misc_feature (20)..(20): Xaa can be any naturally occurring amino acid
  misc_feature (31)..(31): Xaa can be any naturally occurring amino acid
  misc_feature (35)..(35): Xaa can be any naturally occurring amino acid
  misc_feature (48)..(48): Xaa can be any naturally occurring amino acid
  misc_feature (50)..(50): Xaa can be any naturally occurring amino acid
  misc_feature (59)..(59): Xaa can be any naturally occurring amino acid
  misc_feature (67)..(67): Xaa can be any naturally occurring amino acid
  misc_feature (70)..(70): Xaa can be any naturally occurring amino acid
  misc_feature (74)..(74): Xaa can be any naturally occurring amino acid
  misc_feature (79)..(79): Xaa can be any naturally occurring amino acid
  misc_feature (98)..(98): Xaa can be any naturally occurring amino acid
  misc_feature (101)..(101): Xaa can be any naturally occurring amino acid
QVQLVQSGAEVKKPGASVKXSCKASGYTFTXYTMXWVRQAPGQGLEWXGXINPSSGYTXYAQKFQGXVTXTADXSTSTXYMELSSLRSEDTAVYYCAXGDXYVAYWGQGTLVTVSS

SEQ ID NO: 430 - protein, 108 aa, Artificial Sequence
  Synthetic peptide
  misc_feature (1)..(1): Xaa can be any naturally occurring amino acid
  misc_feature (3)..(4): Xaa can be any naturally occurring amino acid
  misc_feature (9)..(11): Xaa can be any naturally occurring amino acid
  misc_feature (15)..(15): Xaa can be any naturally occurring amino acid
  misc_feature (17)..(17): Xaa can be any naturally occurring amino acid
  misc_feature (21)..(21): Xaa can be any naturally occurring amino acid
  misc_feature (24)..(24): Xaa can be any naturally occurring amino acid
  misc_feature (27)..(27): Xaa can be any naturally occurring amino acid
  misc_feature (29)..(29): Xaa can be any naturally occurring amino acid
  misc_feature (32)..(32): Xaa can be any naturally occurring amino acid
  misc_feature (34)..(35): Xaa can be any naturally occurring amino acid
  misc_feature (43)..(44): Xaa can be any naturally occurring amino acid
  misc_feature (48)..(48): Xaa can be any naturally occurring amino acid
  misc_feature (51)..(56): Xaa can be any naturally occurring amino acid
  misc_feature (61)..(61): Xaa can be any naturally occurring amino acid
  misc_feature (67)..(67): Xaa can be any naturally occurring amino acid
  misc_feature (71)..(73): Xaa can be any naturally occurring amino acid
  misc_feature (79)..(81): Xaa can be any naturally occurring amino acid
  misc_feature (84)..(84): Xaa can be any naturally occurring amino acid
  misc_feature (90)..(91): Xaa can be any naturally occurring amino acid
  misc_feature (93)..(96): Xaa can be any naturally occurring amino acid
  misc_feature (101)..(101): Xaa can be any naturally occurring amino acid
  misc_feature (107)..(107): Xaa can be any naturally occurring amino acid
XIXXTQSPXXXSASXGXRVTXTCXASXSXSSXYXXWYQQKPGXXPKLXIYXXXXXXSGVPXRFSGSXSGTXXXLTISSXXXEDXATYYCXXYXXXXLTFGXGTKLEXK

SEQ ID NO: 431 - protein, 108 aa, Artificial Sequence
  Synthetic peptide
  misc_feature (4)..(4): Xaa can be any naturally occurring amino acid
  misc_feature (21)..(21): Xaa can be any naturally occurring amino acid
  misc_feature (32)..(32): Xaa can be any naturally occurring amino acid
  misc_feature (34)..(34): Xaa can be any naturally occurring amino acid
  misc_feature (48)..(48): Xaa can be any naturally occurring amino acid
  misc_feature (51)..(51): Xaa can be any naturally occurring amino acid
  misc_feature (53)..(53): Xaa can be any naturally occurring amino acid
  misc_feature (61)..(61): Xaa can be any naturally occurring amino acid
  misc_feature (67)..(67): Xaa can be any naturally occurring amino acid
  misc_feature (79)..(79): Xaa can be any naturally occurring amino acid
  misc_feature (84)..(84): Xaa can be any naturally occurring amino acid
  misc_feature (91)..(91): Xaa can be any naturally occurring amino acid
  misc_feature (93)..(93): Xaa can be any naturally occurring amino acid
DIQXTQSPSSLSASVGDRVTXTCTASSSVSSXYXHWYQQKPGKAPKLXIYXTXNLASGVPXRFSGSXSGTDYTLTISSXQPEDXATYYCHXYXRSPLTFGQGTKLEIK

SEQ ID NO: 432 - protein, 117 aa, Artificial Sequence
  Synthetic peptide
  misc_feature (3)..(3): Xaa can be any naturally occurring amino acid
  misc_feature (5)..(5): Xaa can be any naturally occurring amino acid
  misc_feature (18)..(19): Xaa can be any naturally occurring amino acid
  misc_feature (23)..(23): Xaa can be any naturally occurring amino acid
  misc_feature (31)..(31): Xaa can be any naturally occurring amino acid
  misc_feature (33)..(33): Xaa can be any naturally occurring amino acid
  misc_feature (35)..(35): Xaa can be any naturally occurring amino acid
  misc_feature (40)..(40): Xaa can be any naturally occurring amino acid
  misc_feature (42)..(42): Xaa can be any naturally occurring amino acid
  misc_feature (49)..(50): Xaa can be any naturally occurring amino acid
  misc_feature (52)..(59): Xaa can be any naturally occurring amino acid
  misc_feature (61)..(61): Xaa can be any naturally occurring amino acid
  misc_feature (64)..(64): Xaa can be any naturally occurring amino acid
  misc_feature (76)..(76): Xaa can be any naturally occurring amino acid
  misc_feature (79)..(81): Xaa can be any naturally occurring amino acid
  misc_feature (87)..(87): Xaa can be any naturally occurring amino acid
  misc_feature (94)..(95): Xaa can be any naturally occurring amino acid
  misc_feature (99)..(99): Xaa can be any naturally occurring amino acid
  misc_feature (106)..(106): Xaa can be any naturally occurring amino acid
  misc_feature (112)..(112): Xaa can be any naturally occurring amino acid
  misc_feature (114)..(114): Xaa can be any naturally occurring amino acid
EVXLXESGGGLVQPGGSXXLSCXASGFTFSXYXMXWVRQXPXKGLEWVXXIXXXXXXXXTXYAXSVKGRFTISRDXSKXXXYLQMNXLRAEDTXXYYCXDGPPSGXWGQGTXLXVSS

SEQ ID NO: 433 - protein, 117 aa, Artificial Sequence
  Synthetic peptide
  misc_feature (31)..(31): Xaa can be any naturally occurring amino acid
  misc_feature (35)..(35): Xaa can be any naturally occurring amino acid
  misc_feature (50)..(50): Xaa can be any naturally occurring amino acid
  misc_feature (55)..(55): Xaa can be any naturally occurring amino acid
  misc_feature (79)..(79): Xaa can be any naturally occurring amino acid
  misc_feature (99)..(99): Xaa can be any naturally occurring amino acid
  misc_feature (106)..(106): Xaa can be any naturally occurring amino acid
EVQLLESGGGLVQPGGSMRLSCAASGFTFSXYWMXWVRQAPGKGLEWVAXIRLKXDNYATHYADSVKGRFTISRDDSKXTVYLQMNSLRAEDTGVYYCXDGPPSGXWGQGTLLTVSS

SEQ ID NO: 434 - protein, 107 aa, Artificial Sequence
  Synthetic peptide
  misc_feature (9)..(9): Xaa can be any naturally occurring amino acid
  misc_feature (17)..(18): Xaa can be any naturally occurring amino acid
  misc_feature (25)..(25): Xaa can be any naturally occurring amino acid
  misc_feature (27)..(28): Xaa can be any naturally occurring amino acid
  misc_feature (30)..(30): Xaa can be any naturally occurring amino acid
  misc_feature (34)..(34): Xaa can be any naturally occurring amino acid
  misc_feature (40)..(40): Xaa can be any naturally occurring amino acid
  misc_feature (43)..(43): Xaa can be any naturally occurring amino acid
  misc_feature (45)..(45): Xaa can be any naturally occurring amino acid
  misc_feature (48)..(48): Xaa can be any naturally occurring amino acid
  misc_feature (50)..(50): Xaa can be any naturally occurring amino acid
  misc_feature (52)..(53): Xaa can be any naturally occurring amino acid
  misc_feature (55)..(56): Xaa can be any naturally occurring amino acid
  misc_feature (70)..(70): Xaa can be any naturally occurring amino acid
  misc_feature (72)..(72): Xaa can be any naturally occurring amino acid
  misc_feature (74)..(74): Xaa can be any naturally occurring amino acid
  misc_feature (76)..(76): Xaa can be any naturally occurring amino acid
  misc_feature (84)..(85): Xaa can be any naturally occurring amino acid
  misc_feature (90)..(91): Xaa can be any naturally occurring amino acid
  misc_feature (93)..(94): Xaa can be any naturally occurring amino acid
  misc_feature (97)..(97): Xaa can be any naturally occurring amino acid
  misc_feature (100)..(100): Xaa can be any naturally occurring amino acid
DIQMTQSPXSLSASVGXXVTITCRXSXXIXSYLXWYQQKXGKXPXLLXYXAXXLXXGVPSRFSGSGSGTXFXLXIXSLQPEDFXXYYCQXXYXXPWXFGXGTKLEIK

SEQ ID NO: 435 - protein, 107 aa, Artificial Sequence
  Synthetic peptide
  misc_feature (25)..(25): Xaa can be any naturally occurring amino acid
  misc_feature (34)..(34): Xaa can be any naturally occurring amino acid
  misc_feature (48)..(48): Xaa can be any naturally occurring amino acid
  misc_feature (53)..(53): Xaa can be any naturally occurring amino acid
  misc_feature (55)..(55): Xaa can be any naturally occurring amino acid
  misc_feature (84)..(85): Xaa can be any naturally occurring amino acid
  misc_feature (90)..(90): Xaa can be any naturally occurring amino acid
  misc_feature (93)..(93): Xaa can be any naturally occurring amino acid
DIQMTQSPSSLSASVGDRVTITCRXSENIYSYLXWYQQKPGKAPKLLXYNAKXLXEGVPSRFSGSGSGTDFTLTISSLQPEDFXXYYCQXHYXVPWTFGQGTKLEIK

SEQ ID NO: 436 - protein, 117 aa, Artificial Sequence
  Synthetic peptide
  misc_feature (5)..(5): Xaa can be any naturally occurring amino acid
  misc_feature (11)..(13): Xaa can be any naturally occurring amino acid
  misc_feature (20)..(20): Xaa can be any naturally occurring amino acid
  misc_feature (29)..(29): Xaa can be any naturally occurring amino acid
  misc_feature (31)..(31): Xaa can be any naturally occurring amino acid
  misc_feature (33)..(33): Xaa can be any naturally occurring amino acid
  misc_feature (37)..(38): Xaa can be any naturally occurring amino acid
  misc_feature (40)..(40): Xaa can be any naturally occurring amino acid
  misc_feature (45)..(45): Xaa can be any naturally occurring amino acid
  misc_feature (48)..(48): Xaa can be any naturally occurring amino acid
  misc_feature (50)..(50): Xaa can be any naturally occurring amino acid
  misc_feature (55)..(57): Xaa can be any naturally occurring amino acid
  misc_feature (59)..(59): Xaa can be any naturally occurring amino acid
  misc_feature (61)..(62): Xaa can be any naturally occurring amino acid
  misc_feature (65)..(68): Xaa can be any naturally occurring amino acid
  misc_feature (70)..(70): Xaa can be any naturally occurring amino acid
  misc_feature (72)..(72): Xaa can be any naturally occurring amino acid
  misc_feature (74)..(74): Xaa can be any naturally occurring amino acid
  misc_feature (76)..(76): Xaa can be any naturally occurring amino acid
  misc_feature (79)..(79): Xaa can be any naturally occurring amino acid
  misc_feature (82)..(82): Xaa can be any naturally occurring amino acid
  misc_feature (84)..(84): Xaa can be any naturally occurring amino acid
  misc_feature (87)..(87): Xaa can be any naturally occurring amino acid
  misc_feature (91)..(91): Xaa can be any naturally occurring amino acid
  misc_feature (97)..(97): Xaa can be any naturally occurring amino acid
  misc_feature (101)..(101): Xaa can be any naturally occurring amino acid
  misc_feature (117)..(117): Xaa can be any naturally occurring amino acid
QVQLXQSGAEXXXPGASVKXSCKASGYTXTXYXMHWXXQXPGQGXEWXGXINPSXXXTXYXXKFXXXXTXTXDXSXSTXYMXLXSLXSEDXAVYYCXRGEXGGFAYWGQGTLVTVSX

SEQ ID NO: 437 - protein, 117 aa, Artificial Sequence
  Synthetic peptide
  misc_feature (20)..(20): Xaa can be any naturally occurring amino acid
  misc_feature (29)..(29): Xaa can be any naturally occurring amino acid
  misc_feature (31)..(31): Xaa can be any naturally occurring amino acid
  misc_feature (37)..(37): Xaa can be any naturally occurring amino acid
  misc_feature (45)..(45): Xaa can be any naturally occurring amino acid
  misc_feature (48)..(48): Xaa can be any naturally occurring amino acid
  misc_feature (56)..(56): Xaa can be any naturally occurring amino acid
  misc_feature (59)..(59): Xaa can be any naturally occurring amino acid
  misc_feature (61)..(62): Xaa can be any naturally occurring amino acid
  misc_feature (65)..(66): Xaa can be any naturally occurring amino acid
  misc_feature (68)..(68): Xaa can be any naturally occurring amino acid
  misc_feature (70)..(70): Xaa can be any naturally occurring amino acid
  misc_feature (74)..(74): Xaa can be any naturally occurring amino acid
  misc_feature (79)..(79): Xaa can be any naturally occurring amino acid
  misc_feature (84)..(84): Xaa can be any naturally occurring amino acid
  misc_feature (97)..(97): Xaa can be any naturally occurring amino acid
  misc_feature (101)..(101): Xaa can be any naturally occurring amino acid
QVQLVQSGAEVKKPGASVKXSCKASGYTXTXYTMHWXRQAPGQGXEWXGYINPSSXYTXYXXKFXXRXTXTADXSTSTXYMELXSLRSEDTAVYYCXRGEXGGFAYWGQGTLVTVSS

SEQ ID NO: 438 - protein, 112 aa, Artificial Sequence
  Synthetic peptide
  misc_feature (7)..(7): Xaa can be any naturally occurring amino acid
  misc_feature (14)..(14): Xaa can be any naturally occurring amino acid
  misc_feature (17)..(18): Xaa can be any naturally occurring amino acid
  misc_feature (31)..(31): Xaa can be any naturally occurring amino acid
  misc_feature (33)..(33): Xaa can be any naturally occurring amino acid
  misc_feature (39)..(39): Xaa can be any naturally occurring amino acid
  misc_feature (41)..(42): Xaa can be any naturally occurring amino acid
  misc_feature (44)..(44): Xaa can be any naturally occurring amino acid
  misc_feature (50)..(51): Xaa can be any naturally occurring amino acid
  misc_feature (55)..(55): Xaa can be any naturally occurring amino acid
  misc_feature (57)..(57): Xaa can be any naturally occurring amino acid
  misc_feature (81)..(81): Xaa can be any naturally occurring amino acid
  misc_feature (88)..(88): Xaa can be any naturally occurring amino acid
  misc_feature (92)..(92): Xaa can be any naturally occurring amino acid
  misc_feature (94)..(96): Xaa can be any naturally occurring amino acid
  misc_feature (99)..(100): Xaa can be any naturally occurring amino acid
  misc_feature (105)..(105): Xaa can be any naturally occurring amino acid
DVVMTQXPLSLPVXLGXXASISCRSSQSLVXSXGNTYLXWXXQXPGQSPXXNPSXTXTHYSGVPDRFSGSGSGTDFTLKIXRVEAEDXGVYXCXXXTHXXYTFGXGTKLEIK

SEQ ID NO: 439 - protein, 112 aa, Artificial Sequence
  Synthetic peptide
  misc_feature (33)..(33): Xaa can be any naturally occurring amino acid
  misc_feature (39)..(39): Xaa can be any naturally occurring amino acid
  misc_feature (55)..(55): Xaa can be any naturally occurring amino acid
  misc_feature (57)..(57): Xaa can be any naturally occurring amino acid
  misc_feature (81)..(81): Xaa can be any naturally occurring amino acid
  misc_feature (95)..(96): Xaa can be any naturally occurring amino acid
DVVMTQSPLSLPVTLGQPASISCRSSQSLVHSXGNTYLXWYQQRPGQSPRLLIYXVXNRFSGVPDRFSGSGSGTDFTLKIXRVEAEDVGVYYCSXXTHVPYTFGQGTKLEIK

SEQ ID NO: 440 - protein, 120 aa, Artificial Sequence
  Synthetic peptide
  misc_feature (5)..(5): Xaa can be any naturally occurring amino acid
  misc_feature (9)..(9): Xaa can be any naturally occurring amino acid
  misc_feature (11)..(12): Xaa can be any naturally occurring amino acid
  misc_feature (20)..(20): Xaa can be any naturally occurring amino acid
  misc_feature (38)..(38): Xaa can be any naturally occurring amino acid
  misc_feature (40)..(41): Xaa can be any naturally occurring amino acid
  misc_feature (43)..(44): Xaa can be any naturally occurring amino acid
  misc_feature (48)..(48): Xaa can be any naturally occurring amino acid
  misc_feature (61)..(61): Xaa can be any naturally occurring amino acid
  misc_feature (65)..(65): Xaa can be any naturally occurring amino acid
  misc_feature (67)..(68): Xaa can be any naturally occurring amino acid
  misc_feature (70)..(70): Xaa can be any naturally occurring amino acid
  misc_feature (72)..(72): Xaa can be any naturally occurring amino acid
  misc_feature (74)..(74): Xaa can be any naturally occurring amino acid
  misc_feature (76)..(76): Xaa can be any naturally occurring amino acid
  misc_feature (79)..(79): Xaa can be any naturally occurring amino acid
  misc_feature (82)..(82): Xaa can be any naturally occurring amino acid
  misc_feature (84)..(84): Xaa can be any naturally occurring amino acid
  misc_feature (87)..(87): Xaa can be any naturally occurring amino acid
  misc_feature (91)..(91): Xaa can be any naturally occurring amino acid
  misc_feature (116)..(116): Xaa can be any naturally occurring amino acid
QVQLXQSGXEXXKPGASVKXSCKASGYSFTGYNMNWVXQXXGXXLEWXGNIDPYYGGSTYXQKFXGXXTXTXDXSXSTXYMXLXSLXSEDXAVYYCARERSGYVFSAMDYWGQGTXVTVS

SEQ ID NO: 441 - protein, 120 aa, Artificial Sequence
  Synthetic peptide
  misc_feature (20)..(20): Xaa can be any naturally occurring amino acid
  misc_feature (48)..(48): Xaa can be any naturally occurring amino acid
  misc_feature (68)..(68): Xaa can be any naturally occurring amino acid
  misc_feature (70)..(70): Xaa can be any naturally occurring amino acid
  misc_feature (79)..(79): Xaa can be any naturally occurring amino acid
QVQLVQSGAEVKKPGASVKXSCKASGYSFTGYNMNWVRQAPGQGLEWXGNIDPYYGGSTYAQKFQGRXTXTRDTSTSTXYMELSSLRSEDTAVYYCARERSGYVFSAMDYWGQGTLVTVS

SEQ ID NO: 442 - protein, 112 aa, Artificial Sequence
  Synthetic peptide
  misc_feature (1)..(1): Xaa can be any naturally occurring amino acid
  misc_feature (3)..(3): Xaa can be any naturally occurring amino acid
  misc_feature (9)..(9): Xaa can be any naturally occurring amino acid
  misc_feature (15)..(15): Xaa can be any naturally occurring amino acid
  misc_feature (18)..(19): Xaa can be any naturally occurring amino acid
  misc_feature (21)..(22): Xaa can be any naturally occurring amino acid
  misc_feature (49)..(49): Xaa can be any naturally occurring amino acid
  misc_feature (51)..(51): Xaa can be any naturally occurring amino acid
  misc_feature (69)..(69): Xaa can be any naturally occurring amino acid
  misc_feature (78)..(78): Xaa can be any naturally occurring amino acid
  misc_feature (84)..(84): Xaa can be any naturally occurring amino acid
  misc_feature (93)..(93): Xaa can be any naturally occurring amino acid
  misc_feature (105)..(105): Xaa can be any naturally occurring amino acid
  misc_feature (111)..(111): Xaa can be any naturally occurring amino acid
XIXMTQSPXSLAVSXGEXXTXXCKSSQSVLFSSNQKNYLAWYQQKPGQXPXLLIYWASTRESGVPDRFXGSGSGTDFXLTISSXQAEDVAVYXCHQYLSSRTFGXGTKLEXK

SEQ ID NO: 443 - protein, 112 aa, Artificial Sequence
  Synthetic peptide
  misc_feature (19)..(19): Xaa can be any naturally occurring amino acid
  misc_feature (21)..(21): Xaa can be any naturally occurring amino acid
  misc_feature (84)..(84): Xaa can be any naturally occurring amino acid
DIVMTQSPDSLAVSLGERXTXNCKSSQSVLFSSNQKNYLAWYQQKPGQPPKLLIYWASTRESGVPDRFSGSGSGTDFTLTISSXQAEDVAVYYCHQYLSSRTFGQGTKLEIK

SEQ ID NO: 444 - protein, 117 aa, Artificial Sequence
  Synthetic peptide
  misc_feature (1)..(1): Xaa can be any naturally occurring amino acid
  misc_feature (5)..(5): Xaa can be any naturally occurring amino acid
  misc_feature (9)..(9): Xaa can be any naturally occurring amino acid
  misc_feature (11)..(12): Xaa can be any naturally occurring amino acid
  misc_feature (20)..(20): Xaa can be any naturally occurring amino acid
  misc_feature (38)..(38): Xaa can be any naturally occurring amino acid
  misc_feature (40)..(41): Xaa can be any naturally occurring amino acid
  misc_feature (43)..(44): Xaa can be any naturally occurring amino acid
  misc_feature (48)..(48): Xaa can be any naturally occurring amino acid
  misc_feature (61)..(61): Xaa can be any naturally occurring amino acid
  misc_feature (63)..(63): Xaa can be any naturally occurring amino acid
  misc_feature (65)..(65): Xaa can be any naturally occurring amino acid
  misc_feature (67)..(67): Xaa can be any naturally occurring amino acid
  misc_feature (69)..(70): Xaa can be any naturally occurring amino acid
  misc_feature (72)..(74): Xaa can be any naturally occurring amino acid
  misc_feature (76)..(76): Xaa can be any naturally occurring amino acid
  misc_feature (79)..(79): Xaa can be any naturally occurring amino acid
  misc_feature (84)..(84): Xaa can be any naturally occurring amino acid
  misc_feature (87)..(87): Xaa can be any naturally occurring amino acid
  misc_feature (91)..(91): Xaa can be any naturally occurring amino acid
  misc_feature (93)..(93): Xaa can be any naturally occurring amino acid
  misc_feature (112)..(113): Xaa can be any naturally occurring amino acid
XVQLXQSGXEXXKPGASVKXSCKASGYRFTDYNMHWVXQXXGXXLEWXGYINPNNGGTNYXQXFXGXVXXTXXXSXSTXYMELXSLXSEDXAXYYCARDYLYFFDCWGQGTXXTVSS

SEQ ID NO: 445 - protein, 107 aa, Artificial Sequence
  Synthetic peptide
  misc_feature (9)..(9): Xaa can be any naturally occurring amino acid
  misc_feature (11)..(11): Xaa can be any naturally occurring amino acid
  misc_feature (15)..(15): Xaa can be any naturally occurring amino acid
  misc_feature (17)..(18): Xaa can be any naturally occurring amino acid
  misc_feature (43)..(43): Xaa can be any naturally occurring amino acid
  misc_feature (45)..(45): Xaa can be any naturally occurring amino acid
  misc_feature (70)..(70): Xaa can be any naturally occurring amino acid
  misc_feature (72)..(74): Xaa can be any naturally occurring amino acid
  misc_feature (80)..(80): Xaa can be any naturally occurring amino acid
  misc_feature (84)..(85): Xaa can be any naturally occurring amino acid
  misc_feature (100)..(100): Xaa can be any naturally occurring amino acid
DIQMTQSPXSXSASXGXXVTITCLASQTIGTWLAWYQQKPGKXPXLLIYAAASLADGVPSRFSGSGSGTXFXXXISSLQXEDFXXYYCQQLYSIPRTFGXGTKLEIK

SEQ ID NO: 446 - protein, 107 aa, Artificial Sequence
  Synthetic peptide
  misc_feature (1)..(1): Xaa can be any naturally occurring amino acid
  misc_feature (15)..(15): Xaa can be any naturally occurring amino acid
  misc_feature (18)..(19): Xaa can be any naturally occurring amino acid
  misc_feature (42)..(42): Xaa can be any naturally occurring amino acid
  misc_feature (49)..(49): Xaa can be any naturally occurring amino acid
  misc_feature (63)..(63): Xaa can be any naturally occurring amino acid
  misc_feature (75)..(76): Xaa can be any naturally occurring amino acid
  misc_feature (78)..(78): Xaa can be any naturally occurring amino acid
  misc_feature (80)..(80): Xaa can be any naturally occurring amino acid
  misc_feature (84)..(84): Xaa can be any naturally occurring amino acid
  misc_feature (88)..(88): Xaa can be any naturally occurring amino acid
  misc_feature (93)..(93): Xaa can be any naturally occurring amino acid
XVQLVESGGGLVQPXGSXXLSCAASGFTFSSFGMHWVRQAPXKGLEWVXYISSDSRTIYYADXVKGRFTISRDNXXNXLXLQMXSLRXEDTAXYYCARDYGRTYEAY

SEQ ID NO: 447 - protein, 111 aa, Artificial Sequence
  Synthetic peptide
  misc_feature (4)..(4): Xaa can be any naturally occurring amino acid
  misc_feature (9)..(9): Xaa can be any naturally occurring amino acid
  misc_feature (17)..(17): Xaa can be any naturally occurring amino acid
  misc_feature (22)..(22): Xaa can be any naturally occurring amino acid
  misc_feature (64)..(64): Xaa can be any naturally occurring amino acid
  misc_feature (78)..(78): Xaa can be any naturally occurring amino acid
  misc_feature (80)..(84): Xaa can be any naturally occurring amino acid
  misc_feature (87)..(87): Xaa can be any naturally occurring amino acid
  misc_feature (89)..(89): Xaa can be any naturally occurring amino acid
  misc_feature (104)..(104): Xaa can be any naturally occurring amino acid
  misc_feature (110)..(110): Xaa can be any naturally occurring amino acid
DIVXTQSPXSLAVSLGXRATIXCRASKSVSTSGYSYIHWYQQKPGQPPKLLIYLASNLESGVPXRFSGSGSGTDFTLXIXXXXXEDXAXYYCQHSRELPLTFGXGTKLEXK

SEQ ID NO: 448 - protein, 111 aa, Artificial Sequence
  Synthetic peptide
  misc_feature (4)..(4): Xaa can be any naturally occurring amino acid
  misc_feature (82)..(82): Xaa can be any naturally occurring amino acid
  misc_feature (110)..(110): Xaa can be any naturally occurring amino acid
DIVXTQSPDSLAVSLGERATINCRASKSVSTSGYSYIHWYQQKPGQPPKLLIYLASNLESGVPDRFSGSGSGTDFTLTISSXQAEDVAVYYCQHSRELPLTFGQGTKLEXK

SEQ ID NO: 449 - protein, 7 aa, Artificial Sequence
  Synthetic peptide
  MISC_FEATURE (6)..(6): Xaa is T, V, F, or D
SSVSSXY

SEQ ID NO: 450 - protein, 3 aa, Artificial Sequence
  Synthetic peptide
  MISC_FEATURE (1)..(1): Xaa is S, T, Q, or  A
  MISC_FEATURE (3)..(3): Xaa is S, T, D, or Q
XTX

SEQ ID NO: 451 - protein, 9 aa, Artificial Sequence
  Synthetic peptide
  MISC_FEATURE (2)..(2): Xaa is Q, H or S
  MISC_FEATURE (4)..(4): Xaa is H, Y, Q, or S
HXYXRSPLT

SEQ ID NO: 452 - protein, 7 aa, Artificial Sequence
  Synthetic peptide
  MISC_FEATURE (5)..(5): Xaa is T, V, D, or S
YTFTXYT

SEQ ID NO: 453 - protein, 9 aa, Artificial Sequence
  Synthetic peptide
  MISC_FEATURE (2)..(2): Xaa is N, Q, H, D, S, R, or A
AXGDYYVAY

SEQ ID NO: 454 - protein, 9 aa, Artificial Sequence
  Synthetic peptide
  MISC_FEATURE (2)..(2): Xaa is H, Q, S, or T
  MISC_FEATURE (5)..(5): Xaa is T, S, N, or G
QXHYXVPWT

SEQ ID NO: 455 - protein, 7 aa, Artificial Sequence
  Synthetic peptide
  MISC_FEATURE (5)..(5): Xaa is N, S, R, q, s, or a
  MISC_FEATURE (7)..(7): Xaa is w, h, y, or f
FTFSXYX

SEQ ID NO: 456 - protein, 10 aa, Artificial Sequence
  Synthetic peptide
  MISC_FEATURE (5)..(5): Xaa is S, N, A, or T
  MISC_FEATURE (7)..(7): Xaa is Q, S,A, or N
IRLKXDXYAT

SEQ ID NO: 457 - protein, 8 aa, Artificial Sequence
  Synthetic peptide
  MISC_FEATURE (1)..(1): Xaa is N, D, A, or T
  MISC_FEATURE (8)..(8): Xaa is S, T, A, C, Y
XDGPPSGX

SEQ ID NO: 458 - protein, 11 aa, Artificial Sequence
  Synthetic peptide
  MISC_FEATURE (7)..(7): Xaa is D, N, E, Q, S, or A
  MISC_FEATURE (9)..(9): Xaa is Q, S, A, D, or N
QSLVHSXGXTY

SEQ ID NO: 459 - protein, 3 aa, Artificial Sequence
  Synthetic peptide
  MISC_FEATURE (1)..(1): Xaa is K, Q, or R
  MISC_FEATURE (3)..(3): Xaa is S, T, or V
XVX

SEQ ID NO: 460 - protein, 9 aa, Artificial Sequence
  Synthetic peptide
  MISC_FEATURE (2)..(2): Xaa is Q, H, or T
  MISC_FEATURE (3)..(3): Xaa is S, G, T, or D
SXXTHVPYT

SEQ ID NO: 461 - protein, 9 aa, Artificial Sequence
  Synthetic peptide
  MISC_FEATURE (3)..(3): Xaa is F, Y, S, or T
  MISC_FEATURE (5)..(5): Xaa is S, T, Y , or D
YTXTXYTMH

SEQ ID NO: 462 - protein, 8 aa, Artificial Sequence
  Synthetic peptide
  MISC_FEATURE (2)..(2): Xaa is Q, S, A, or N
  MISC_FEATURE (6)..(6): Xaa is T, S, V, D, or G
IXPSSXYT

SEQ ID NO: 463 - protein, 10 aa, Artificial Sequence
  Synthetic peptide
  MISC_FEATURE (1)..(1): Xaa is S, A, T, or V
  MISC_FEATURE (5)..(5): Xaa is L, V, or F
XRGEXGGFAY

SEQ ID NO: 464 - protein, 6 aa, Artificial Sequence
  Synthetic peptide
  MISC_FEATURE (6)..(6): Xaa is W, H, Y, or F
QTIGYX

SEQ ID NO: 465 - protein, 8 aa, Artificial Sequence
  Synthetic peptide
  MISC_FEATURE (3)..(3): Xaa is R or T
  MISC_FEATURE (8)..(8): Xaa is N, Q, S, or A
GYXFTDYX

SEQ ID NO: 466 - protein, 8 aa, Artificial Sequence
  Synthetic peptide
  MISC_FEATURE (2)..(2): Xaa is N, Q, S, or A
  MISC_FEATURE (4)..(4): Xaa is N, Q, S, or A
  MISC_FEATURE (5)..(5): Xaa is N, Q, S, or A
IXPXXGGT

SEQ ID NO: 467 - protein, 8 aa, Artificial Sequence
  Synthetic peptide
  MISC_FEATURE (8)..(8): Xaa is C, Y, S, or A
DYLYFFDX

SEQ ID NO: 468 - protein, 8 aa, Artificial Sequence
  Synthetic peptide
  MISC_FEATURE (4)..(4): Xaa is D, E, S, or A
ISSXSRTI

SEQ ID NO: 469 - protein, 9 aa, Artificial Sequence
  Synthetic peptide
DYGRTYEAY

SEQ ID NO: 470 - protein, 12 aa, Artificial Sequence
  Synthetic peptide
  MISC_FEATURE (8)..(8): Xaa is Q, S, A, D, or N
  MISC_FEATURE (11)..(11): Xaa is Q, S, A, D, or N
QSVLFSSXQKXY

SEQ ID NO: 471 - protein, 3 aa, Artificial Sequence
  Synthetic peptide
  MISC_FEATURE (1)..(1): Xaa is H, Y, F, or W
XAS

SEQ ID NO: 472 - protein, 8 aa, Artificial Sequence
  Synthetic peptide
  MISC_FEATURE (8)..(8): Xaa is N, Q, S, or A
GYSFTFYX

SEQ ID NO: 473 - protein, 8 aa, Artificial Sequence
  Synthetic peptide
  MISC_FEATURE (2)..(2): Xaa is A, S, E, or D
IXPYYGGS

SEQ ID NO: 474 - protein, 12 aa, Artificial Sequence
  Synthetic peptide
ERSGYVFSAMDY

SEQ ID NO: 475 - protein, 8 aa, Artificial Sequence
  Synthetic peptide
  MISC_FEATURE (2)..(2): Xaa is Q, S, A, or N
IXPSSGYT

SEQ ID NO: 476 - protein, 6 aa, Artificial Sequence
  Synthetic peptide
  MISC_FEATURE (2)..(2): Xaa is Q, S, A, D, or N
EXIYSY

SEQ ID NO: 477 - protein, 3 aa, Artificial Sequence
  Synthetic peptide
  MISC_FEATURE (1)..(1): Xaa is Q, S, A, D, or N
XAK

SEQ ID NO: 478 - protein, 116 aa, Artificial Sequence
  Synthetic peptide
  MISC_FEATURE (20)..(20): Xaa is M or V
  MISC_FEATURE (31)..(31): Xaa is T, V, D, or S
  MISC_FEATURE (48)..(48): Xaa is I or M
  MISC_FEATURE (52)..(52): Xaa is Q, S, A, or N
  MISC_FEATURE (70)..(70): Xaa is L or M
  MISC_FEATURE (74)..(74): Xaa is T or K
  MISC_FEATURE (98)..(98): Xaa is N, Q, H, D, S, R,or A
QVQLVQSGAEVKKPGASVKXSCKASGYTFTXYTMHWVRQAPGQGLEWXGFIXPSSGYTDYAQKFQGRVTXTADXSTSTVYMELSSLRSEDTAVYYCAXGDYYVAYWGQGTLVTVSS

SEQ ID NO: 479 - protein, 108 aa, Artificial Sequence
  Synthetic peptide
  MISC_FEATURE (4)..(4): Xaa is L or M
  MISC_FEATURE (21)..(21): Xaa is M or I
  MISC_FEATURE (32)..(32): Xaa is T, V, F, or D
  MISC_FEATURE (48)..(48): Xaa is W or L
  MISC_FEATURE (51)..(51): Xaa is S, t, Q or A
  MISC_FEATURE (53)..(53): Xaa is S,T, D or Q
  MISC_FEATURE (79)..(79): Xaa is M or L
  MISC_FEATURE (84)..(84): Xaa is A or F
  MISC_FEATURE (91)..(91): Xaa is Q, H or S
  MISC_FEATURE (93)..(93): Xaa is H, Y, Q, or S
DIQXTQSPSSLSASVGDRVTXTCTASSSVSSXYFHWYQQKPGKAPKLXIYXTXNLASGVPSRFSGSGSGTDYTLTISSXQPEDXATYYCHXYXRSPLTFGQGTKLEIK

SEQ ID NO: 480 - protein, 117 aa, Artificial Sequence
  Synthetic peptide
  MISC_FEATURE (31)..(31): Xaa is N, S, R, Q or A
  MISC_FEATURE (33)..(33): Xaa is W, H, Y or F
  MISC_FEATURE (55)..(55): Xaa is S, N, A, or T
  MISC_FEATURE (57)..(57): Xaa is Q, S, A, or N
  MISC_FEATURE (99)..(99): Xaa is N, D, or T
  MISC_FEATURE (106)..(106): Xaa is S, T, A, C, or Y
EVQLLESGGGLVQPGGSMRLSCAASGFTFSXYXMNWVRQAPGKGLEWVAQIRLKXDXYATHYADSVKGRFTISRDDSKNTVYLQMNSLRAEDTGVYYCXDGPPSGXWGQGTLLTVSS

SEQ ID NO: 481 - protein, 107 aa, Artificial Sequence
  Synthetic peptide
  MISC_FEATURE (28)..(28): Xaa is Q, S, A, D, or N
  MISC_FEATURE (48)..(48): Xaa is V or I
  MISC_FEATURE (50)..(50): Xaa is S, T, Q or A
  MISC_FEATURE (84)..(84): Xaa is G or A
  MISC_FEATURE (90)..(90): Xaa is H, Q, S or T
  MISC_FEATURE (93)..(93): Xaa is T, S, N, or G
DIQMTQSPSSLSASVGDRVTITCRISEXIYSYLAWYQQKPGKAPKLLXYXAKILVEGVPSRFSGSGSGTDFTLTISSLQPEDFXTYYCQXHYXVPWTFGQGTKLEIK

SEQ ID NO: 482 - protein, 117 aa, Artificial Sequence
  Synthetic peptide
  MISC_FEATURE (20)..(20): Xaa is M or V
  MISC_FEATURE (29)..(29): Xaa is F, Y, S or T
  MISC_FEATURE (31)..(31): Xaa is S, T, Y, or D
  MISC_FEATURE (37)..(37): Xaa is I or V
  MISC_FEATURE (45)..(45): Xaa is Q or L
  MISC_FEATURE (48)..(48): Xaa is I or M
  MISC_FEATURE (52)..(52): Xaa is Q, S, A, or N
  MISC_FEATURE (56)..(56): Xaa is T, S, V, D or G
  MISC_FEATURE (61)..(61): Xaa is I or A
  MISC_FEATURE (62)..(62): Xaa is K or Q
  MISC_FEATURE (65)..(65): Xaa is K or Q
  MISC_FEATURE (66)..(66): Xaa is D or G
  MISC_FEATURE (68)..(68): Xaa is A or V
  MISC_FEATURE (70)..(70): Xaa is L or M
  MISC_FEATURE (74)..(74): Xaa is T or K
  MISC_FEATURE (79)..(79): Xaa is A or V
  MISC_FEATURE (97)..(97): Xaa is S, A, T, or V
  MISC_FEATURE (101)..(97): Xaa is L, V, or F
  misc_feature (101)..(101): Xaa can be any naturally occurring amino acid
QVQLVQSGAEVKKPGASVKXSCKASGYTXTXYTMHWXRQAPGQGXEWXGYIXPSSXYTHYXXKFXXRXTXTADXSTSTXYMELSSLRSEDTAVYYCXRGEXGGFAYWGQGTLVTVSS

SEQ ID NO: 483 - protein, 112 aa, Artificial Sequence
  Synthetic peptide
  MISC_FEATURE (33)..(33): Xaa is D, N, E, Q, S, or A
  MISC_FEATURE (35)..(35): Xaa is Q, S, A, D, or N
  MISC_FEATURE (55)..(55): Xaa is K, Q, or R
  MISC_FEATURE (57)..(57): Xaa is S, T, or V
  MISC_FEATURE (95)..(95): Xaa is Q, H, or T
  MISC_FEATURE (96)..(96): Xaa is S, G, T, or D
DVVMTQSPLSLPVTLGQPASISCRSSQSLVHSDGXTYLNWYQQRPGQSPRLLIYXVXNRFSGVPDRFSGSGSGTDFTLKISRVEAEDVGVYYCSXXTHVPYTFGQGTKLEIK

SEQ ID NO: 484 - protein, 121 aa, Artificial Sequence
  Synthetic peptide
  MISC_FEATURE (20)..(20): Xaa is I or V
  MISC_FEATURE (33)..(33): Xaa is N, Q, S, or A
  MISC_FEATURE (48)..(48): Xaa is I or M
  MISC_FEATURE (52)..(52): Xaa is A, S, E or D
  MISC_FEATURE (68)..(68): Xaa is A or V
  MISC_FEATURE (70)..(70): Xaa is L or M
  MISC_FEATURE (79)..(79): Xaa is A or V
QVQLVQSGAEVKKPGASVKXSCKASGYSFTGYXMNWVRQAPGQGLEWXGNIXPYYGGSTYAQKFQGRXTXTVDTSTSTXYMELSSLRSEDTAVYYCARERSGYVFSAMDYWGQGTLVTVSS

SEQ ID NO: 485 - protein, 112 aa, Artificial Sequence
  Synthetic peptide
  MISC_FEATURE (19)..(19): Xaa is V or A
  MISC_FEATURE (21)..(21): Xaa is M or I
  MISC_FEATURE (34)..(34): Xaa is Q, S, A, D, or N
  MISC_FEATURE (37)..(37): Xaa is Q, S, A, D, or N
  MISC_FEATURE (56)..(56): Xaa is H, Y, F, or W
  MISC_FEATURE (84)..(84): Xaa is V or L
DIVMTQSPDSLAVSLGERXTXNCKSSQSVLFSSXQKXYLAWYQQKPGQPPKLLIYXASTRESGVPDRFSGSGSGTDFTLTISSXQAEDVAVYYCHQYLSSRTFGQGTKLEIK

SEQ ID NO: 486 - protein, 118 aa, Artificial Sequence
  Synthetic peptide
  MISC_FEATURE (54)..(54): Xaa is D, E, S, or A
EVQLVESGGGLVQPGGSLRLSCAASGFTFSSFGMHWVRQAPGKGLEWVAYISSXSRTIYYADSVKGRFTISRDNAKNSLYLQMNSLRAEDTAVYYCARDYGRTYEAYWGQGTLVTVSS

SEQ ID NO: 487 - protein, 111 aa, Artificial Sequence
  Synthetic peptide
  MISC_FEATURE (4)..(4): Xaa is M or L
  MISC_FEATURE (82)..(82): Xaa is V or L
  MISC_FEATURE (110)..(110): Xaa is I or L
DIVXTQSPDSLAVSLGERATINCRASKSVSTSGYSYIHWYQQKPGQPPKLLIYLASNLESGVPDRFSGSGSGTDFTLTISSXQAEDVAVYYCQHSRELPLTFGQGTKLEIK

SEQ ID NO: 488 - protein, 117 aa, Artificial Sequence
  Synthetic peptide
  MISC_FEATURE (28)..(28): Xaa is R or T
  MISC_FEATURE (33)..(33): Xaa is N, Q, S or A
  MISC_FEATURE (52)..(52): Xaa is N, Q, S or A
  MISC_FEATURE (54)..(54): Xaa is N, Q, S or A
  MISC_FEATURE (55)..(55): Xaa is N, Q, S, or A
  MISC_FEATURE (106)..(106): Xaa is C, Y, S, or A
QVQLVQSGAEVKKPGASVKMSCKASGYXFTDYXMHWVRQAPGQGLEWIGYIXPXXGGTNYAQKFQGRATLTVDTSTSTAYMELSSLRSEDTAVYYCARDYLYFFDXWGQGTLLTVSS

SEQ ID NO: 489 - protein, 107 aa, Artificial Sequence
  Synthetic peptide
  MISC_FEATURE (24)..(24): Xaa is L or R
  MISC_FEATURE (32)..(32): Xaa is W, H, Y, or F
DIQMTQSPSSLSASVGDRVTITCLASQTIGTXLAWYQQKPGKAPKLLIYAAASLADGVPSRFSGSGSGTDFTFTISSLQPEDFVTYYCQQLYSIPRTFGQGTKLEIK